European Patent Application EP 4 194 556 A1, published June 14, 2023. Title: 一种融合蛋白及其用途. Applicant: 北京中因科技有限公司. The sequence listing filed with the application follows.

SEQUENCE LISTING (55 sequences)

SEQ ID NO: 1 - DNA, 4787 bp, 人工序列（Artificial Sequence）
  pAV-CAG-RdCVF-BGH
cctgcaggcagctgcgcgctcgctcgctcactgaggccgcccgggcgtcgggcgacctttggtcgcccggcctcagtgagcgagcgagcgcgcagagagggagtggccaactccatcactaggggttcctgcggccggtcgcgtctagtactagtctagtcgcgtaccattgacgtcaataatgacgtatgttcccatagtaacgccaatagggactttccattgacgtcaatgggtggagtatttacggtaaactgcccacttggcagtacatcaagtgtatcatatgccaagtacgccccctattgacgtcaatgacggtaaatggcccgcctggcattatgcccagtacatgaccttatgggactttcctacttggcagtacatctacgtattagtcatcgctattaccatggtcgaggtgagccccacgttctgcttcactctccccatctcccccccctccccacccccaattttgtatttatttattttttaattattttgtgcagcgatgggggcggggggggggggggggcgcgcgccaggcggggcggggcggggcgaggggcggggcggggcgaggcggagaggtgcggcggcagccaatcagagcggcgcgctccgaaagtttccttttatggcgaggcggcggcggcggcggccctataaaaagcgaagcgcgcggcgggcgggagtcgctgcgacgctgccttcgccccgtgccccgctccgccgccgcctcgcgccgcccgccccggctctgactgaccgcgttactcccacaggtgagcgggcgggacggcccttctcctccgggctgtaattagcgcttggtttaatgacggcttgtttcttttctgtggctgcgtgaaagccttgaggggctccgggagggccctttgtgcggggggagcggctcggggctgtccgcggggggacggctgccttcgggggggacggggcagggcggggttcggcttctggcgtgtgaccggcggctctagagcctctgctaaccatgttcatgccttcttctttttcctacagctcctgggcaacgtgctggttattgtgctgtctcatcattttggcaaagaattggatcggtaccgaggagatctgccaccatggcctccctgttctctggccgcatcctgatccgcaacaatagcgaccaggacgagctggatacggaggctgaggtcagtcgcaggctggagaaccggctggtgctgctgttctttggtgctggggcttgtccacagtgccaggccttcgtgcccatcctcaaggacttcttcgtgcggctcacagatgagttctatgtactgcgggcggctcagctggccctggtgtacgtgtcccaggactccacggaggagcagcaggacctgttcctcaaggacatgccaaagaaatggcttttcctgccctttgaggatgatctgaggaggtgataaacgcgtctgtgccttctagttgccagccatctgttgtttgcccctcccccgtgccttccttgaccctggaaggtgccactcccactgtcctttcctaataaaatgaggaaattgcatcgcattgtctgagtaggtgtcattctattctggggggtggggtggggcaggacagcaagggggaggattgggaagacaatagcaggcatgctggggatgcggtgggctctatggggtaaccacgtgcggacccaacggccgcaggaacccctagtgatggagttggccactccctctctgcgcgctcgctcgctcactgaggccgggcgaccaaaggtcgcccgacgcccgggctttgcccgggcggcctcagtgagcgagcgagcgcgcagctgcctgcaggggcgcctgatgcggtattttctccttacgcatctgtgcggtatttcacaccgcatacgtcaaagcaaccatagtacgcgccctgtagcggcacattaagcgcggcgggtgtggtggttacgcgcagcgtgaccgctacacttgccagcgccttagcgcccgctcctttcgctttcttcccttcctttctcgccacgttcgccggctttccccgtcaagctctaaatcgggggctccctttagggttccgatttagtgctttacggcacctcgaccccaaaaaacttgatttgggtgatggttcacgtagtgggccatcgccctgatagacggtttttcgccctttgacgttggagtccacgttctttaatagtggactcttgttccaaactggaacaacactcaactctatctcgggctattcttttgatttataagggattttgccgatttcggtctattggttaaaaaatgagctgatttaacaaaaatttaacgcgaattttaacaaaatattaacgtttacaattttatggtgcactctcagtacaatctgctctgatgccgcatagttaagccagccccgacacccgccaacacccgctgacgcgccctgacgggcttgtctgctcccggcatccgcttacagacaagctgtgaccgtctccgggagctgcatgtgtcagaggttttcaccgtcatcaccgaaacgcgcgagacgaaagggcctcgtgatacgcctatttttataggttaatgtcatgataataatggtttcttagacgtcaggtggcacttttcggggaaatgtgcgcggaacccctatttgtttatttttctaaatacattcaaatatgtatccgctcatgagacaataaccctgataaatgcttcaataatattgaaaaaggaagagtcctgaggcggaaagaaccagctgtggaatgtgtgtcagttagggtgtggaaagtccccaggctccccagcaggcagaagtatgcaaagcatgcatctcaattagtcagcaaccaggtgtggaaagtccccaggctccccagcaggcagaagtatgcaaagcatgcatctcaattagtcagcaaccatagtcccgcccctaactccgcccatcccgcccctaactccgcccagttccgcccattctccgccccatggctgactaattttttttatttatgcagaggccgaggccgcctcggcctctgagctattccagaagtagtgaggaggcttttttggaggcctaggcttttgcaaagatcgatcaagagacaggatgaggatcgtttcgcatgattgaacaagatggattgcacgcaggttctccggccgcttgggtggagaggctattcggctatgactgggcacaacagacaatcggctgctctgatgccgccgtgttccggctgtcagcgcaggggcgcccggttctttttgtcaagaccgacctgtccggtgccctgaatgaactgcaagacgaggcagcgcggctatcgtggctggccacgacgggcgttccttgcgcagctgtgctcgacgttgtcactgaagcgggaagggactggctgctattgggcgaagtgccggggcaggatctcctgtcatctcaccttgctcctgccgagaaagtatccatcatggctgatgcaatgcggcggctgcatacgcttgatccggctacctgcccattcgaccaccaagcgaaacatcgcatcgagcgagcacgtactcggatggaagccggtcttgtcgatcaggatgatctggacgaagagcatcaggggctcgcgccagccgaactgttcgccaggctcaaggcgagcatgcccgacggcgaggatctcgtcgtgacccatggcgatgcctgcttgccgaatatcatggtggaaaatggccgcttttctggattcatcgactgtggccggctgggtgtggcggaccgctatcaggacatagcgttggctacccgtgatattgctgaagagcttggcggcgaatgggctgaccgcttcctcgtgctttacggtatcgccgctcccgattcgcagcgcatcgccttctatcgccttcttgacgagttcttctgactgtcagaccaagtttactcatatatactttagattgatttaaaacttcatttttaatttaaaaggatctaggtgaagatcctttttgataatctcatgaccaaaatcccttaacgtgagttttcgttccactgagcgtcagaccccgtagaaaagatcaaaggatcttcttgagatcctttttttctgcgcgtaatctgctgcttgcaaacaaaaaaaccaccgctaccagcggtggtttgtttgccggatcaagagctaccaactctttttccgaaggtaactggcttcagcagagcgcagataccaaatactgttcttctagtgtagccgtagttaggccaccacttcaagaactctgtagcaccgcctacatacctcgctctgctaatcctgttaccagtggctgctgccagtggcgataagtcgtgtcttaccgggttggactcaagacgatagttaccggataaggcgcagcggtcgggctgaacggggggttcgtgcacacagcccagcttggagcgaacgacctacaccgaactgagatacctacagcgtgagctatgagaaagcgccacgcttcccgaagggagaaaggcggacaggtatccggtaagcggcagggtcggaacaggagagcgcacgagggagcttccagggggaaacgcctggtatctttatagtcctgtcgggtttcgccacctctgacttgagcgtcgatttttgtgatgctcgtcaggggggcggagcctatggaaaaacgccagcaacgcggcctttttacggttcctggccttttgctggccttttgctcacatgt

SEQ ID NO: 2 - DNA, 4835 bp, 人工序列（Artificial Sequence）
  pAV-CAG-spGL-RdCVF-BGH
cctgcaggcagctgcgcgctcgctcgctcactgaggccgcccgggcgtcgggcgacctttggtcgcccggcctcagtgagcgagcgagcgcgcagagagggagtggccaactccatcactaggggttcctgcggccggtcgcgtctagtactagtctagtcgcgtaccattgacgtcaataatgacgtatgttcccatagtaacgccaatagggactttccattgacgtcaatgggtggagtatttacggtaaactgcccacttggcagtacatcaagtgtatcatatgccaagtacgccccctattgacgtcaatgacggtaaatggcccgcctggcattatgcccagtacatgaccttatgggactttcctacttggcagtacatctacgtattagtcatcgctattaccatggtcgaggtgagccccacgttctgcttcactctccccatctcccccccctccccacccccaattttgtatttatttattttttaattattttgtgcagcgatgggggcggggggggggggggggcgcgcgccaggcggggcggggcggggcgaggggcggggcggggcgaggcggagaggtgcggcggcagccaatcagagcggcgcgctccgaaagtttccttttatggcgaggcggcggcggcggcggccctataaaaagcgaagcgcgcggcgggcgggagtcgctgcgacgctgccttcgccccgtgccccgctccgccgccgcctcgcgccgcccgccccggctctgactgaccgcgttactcccacaggtgagcgggcgggacggcccttctcctccgggctgtaattagcgcttggtttaatgacggcttgtttcttttctgtggctgcgtgaaagccttgaggggctccgggagggccctttgtgcggggggagcggctcggggctgtccgcggggggacggctgccttcgggggggacggggcagggcggggttcggcttctggcgtgtgaccggcggctctagagcctctgctaaccatgttcatgccttcttctttttcctacagctcctgggcaacgtgctggttattgtgctgtctcatcattttggcaaagaattggatcggtaccgaggagatctgccaccatgggagtcaaagttctgtttgccctgatctgcatcgctgtggccgaggccgcctccctgttctctggccgcatcctgatccgcaacaatagcgaccaggacgagctggatacggaggctgaggtcagtcgcaggctggagaaccggctggtgctgctgttctttggtgctggggcttgtccacagtgccaggccttcgtgcccatcctcaaggacttcttcgtgcggctcacagatgagttctatgtactgcgggcggctcagctggccctggtgtacgtgtcccaggactccacggaggagcagcaggacctgttcctcaaggacatgccaaagaaatggcttttcctgccctttgaggatgatctgaggaggtgataaacgcgtctgtgccttctagttgccagccatctgttgtttgcccctcccccgtgccttccttgaccctggaaggtgccactcccactgtcctttcctaataaaatgaggaaattgcatcgcattgtctgagtaggtgtcattctattctggggggtggggtggggcaggacagcaagggggaggattgggaagacaatagcaggcatgctggggatgcggtgggctctatggggtaaccacgtgcggacccaacggccgcaggaacccctagtgatggagttggccactccctctctgcgcgctcgctcgctcactgaggccgggcgaccaaaggtcgcccgacgcccgggctttgcccgggcggcctcagtgagcgagcgagcgcgcagctgcctgcaggggcgcctgatgcggtattttctccttacgcatctgtgcggtatttcacaccgcatacgtcaaagcaaccatagtacgcgccctgtagcggcacattaagcgcggcgggtgtggtggttacgcgcagcgtgaccgctacacttgccagcgccttagcgcccgctcctttcgctttcttcccttcctttctcgccacgttcgccggctttccccgtcaagctctaaatcgggggctccctttagggttccgatttagtgctttacggcacctcgaccccaaaaaacttgatttgggtgatggttcacgtagtgggccatcgccctgatagacggtttttcgccctttgacgttggagtccacgttctttaatagtggactcttgttccaaactggaacaacactcaactctatctcgggctattcttttgatttataagggattttgccgatttcggtctattggttaaaaaatgagctgatttaacaaaaatttaacgcgaattttaacaaaatattaacgtttacaattttatggtgcactctcagtacaatctgctctgatgccgcatagttaagccagccccgacacccgccaacacccgctgacgcgccctgacgggcttgtctgctcccggcatccgcttacagacaagctgtgaccgtctccgggagctgcatgtgtcagaggttttcaccgtcatcaccgaaacgcgcgagacgaaagggcctcgtgatacgcctatttttataggttaatgtcatgataataatggtttcttagacgtcaggtggcacttttcggggaaatgtgcgcggaacccctatttgtttatttttctaaatacattcaaatatgtatccgctcatgagacaataaccctgataaatgcttcaataatattgaaaaaggaagagtcctgaggcggaaagaaccagctgtggaatgtgtgtcagttagggtgtggaaagtccccaggctccccagcaggcagaagtatgcaaagcatgcatctcaattagtcagcaaccaggtgtggaaagtccccaggctccccagcaggcagaagtatgcaaagcatgcatctcaattagtcagcaaccatagtcccgcccctaactccgcccatcccgcccctaactccgcccagttccgcccattctccgccccatggctgactaattttttttatttatgcagaggccgaggccgcctcggcctctgagctattccagaagtagtgaggaggcttttttggaggcctaggcttttgcaaagatcgatcaagagacaggatgaggatcgtttcgcatgattgaacaagatggattgcacgcaggttctccggccgcttgggtggagaggctattcggctatgactgggcacaacagacaatcggctgctctgatgccgccgtgttccggctgtcagcgcaggggcgcccggttctttttgtcaagaccgacctgtccggtgccctgaatgaactgcaagacgaggcagcgcggctatcgtggctggccacgacgggcgttccttgcgcagctgtgctcgacgttgtcactgaagcgggaagggactggctgctattgggcgaagtgccggggcaggatctcctgtcatctcaccttgctcctgccgagaaagtatccatcatggctgatgcaatgcggcggctgcatacgcttgatccggctacctgcccattcgaccaccaagcgaaacatcgcatcgagcgagcacgtactcggatggaagccggtcttgtcgatcaggatgatctggacgaagagcatcaggggctcgcgccagccgaactgttcgccaggctcaaggcgagcatgcccgacggcgaggatctcgtcgtgacccatggcgatgcctgcttgccgaatatcatggtggaaaatggccgcttttctggattcatcgactgtggccggctgggtgtggcggaccgctatcaggacatagcgttggctacccgtgatattgctgaagagcttggcggcgaatgggctgaccgcttcctcgtgctttacggtatcgccgctcccgattcgcagcgcatcgccttctatcgccttcttgacgagttcttctgactgtcagaccaagtttactcatatatactttagattgatttaaaacttcatttttaatttaaaaggatctaggtgaagatcctttttgataatctcatgaccaaaatcccttaacgtgagttttcgttccactgagcgtcagaccccgtagaaaagatcaaaggatcttcttgagatcctttttttctgcgcgtaatctgctgcttgcaaacaaaaaaaccaccgctaccagcggtggtttgtttgccggatcaagagctaccaactctttttccgaaggtaactggcttcagcagagcgcagataccaaatactgttcttctagtgtagccgtagttaggccaccacttcaagaactctgtagcaccgcctacatacctcgctctgctaatcctgttaccagtggctgctgccagtggcgataagtcgtgtcttaccgggttggactcaagacgatagttaccggataaggcgcagcggtcgggctgaacggggggttcgtgcacacagcccagcttggagcgaacgacctacaccgaactgagatacctacagcgtgagctatgagaaagcgccacgcttcccgaagggagaaaggcggacaggtatccggtaagcggcagggtcggaacaggagagcgcacgagggagcttccagggggaaacgcctggtatctttatagtcctgtcgggtttcgccacctctgacttgagcgtcgatttttgtgatgctcgtcaggggggcggagcctatggaaaaacgccagcaacgcggcctttttacggttcctggccttttgctggccttttgctcacatgt

SEQ ID NO: 3 - DNA, 4937 bp, 人工序列（Artificial Sequence）
  pAV-CAG-spGUCY2D-RdCVF-BGH
cctgcaggcagctgcgcgctcgctcgctcactgaggccgcccgggcgtcgggcgacctttggtcgcccggcctcagtgagcgagcgagcgcgcagagagggagtggccaactccatcactaggggttcctgcggccggtcgcgtctagtactagtctagtcgcgtaccattgacgtcaataatgacgtatgttcccatagtaacgccaatagggactttccattgacgtcaatgggtggagtatttacggtaaactgcccacttggcagtacatcaagtgtatcatatgccaagtacgccccctattgacgtcaatgacggtaaatggcccgcctggcattatgcccagtacatgaccttatgggactttcctacttggcagtacatctacgtattagtcatcgctattaccatggtcgaggtgagccccacgttctgcttcactctccccatctcccccccctccccacccccaattttgtatttatttattttttaattattttgtgcagcgatgggggcggggggggggggggggcgcgcgccaggcggggcggggcggggcgaggggcggggcggggcgaggcggagaggtgcggcggcagccaatcagagcggcgcgctccgaaagtttccttttatggcgaggcggcggcggcggcggccctataaaaagcgaagcgcgcggcgggcgggagtcgctgcgacgctgccttcgccccgtgccccgctccgccgccgcctcgcgccgcccgccccggctctgactgaccgcgttactcccacaggtgagcgggcgggacggcccttctcctccgggctgtaattagcgcttggtttaatgacggcttgtttcttttctgtggctgcgtgaaagccttgaggggctccgggagggccctttgtgcggggggagcggctcggggctgtccgcggggggacggctgccttcgggggggacggggcagggcggggttcggcttctggcgtgtgaccggcggctctagagcctctgctaaccatgttcatgccttcttctttttcctacagctcctgggcaacgtgctggttattgtgctgtctcatcattttggcaaagaattggatcggtaccgaggagatctgccaccatgaccgcctgtgctagaagagccggcggcctccctgatcctggcctgtgcggccctgcttggtgggccccctccctccctagactcccccgggctctgcctagactccccctcctgctcctgctcctgctgctccaaccccccgccctgagcgcctccctgttctctggccgcatcctgatccgcaacaatagcgaccaggacgagctggatacggaggctgaggtcagtcgcaggctggagaaccggctggtgctgctgttctttggtgctggggcttgtccacagtgccaggccttcgtgcccatcctcaaggacttcttcgtgcggctcacagatgagttctatgtactgcgggcggctcagctggccctggtgtacgtgtcccaggactccacggaggagcagcaggacctgttcctcaaggacatgccaaagaaatggcttttcctgccctttgaggatgatctgaggaggtgataaacgcgtctgtgccttctagttgccagccatctgttgtttgcccctcccccgtgccttccttgaccctggaaggtgccactcccactgtcctttcctaataaaatgaggaaattgcatcgcattgtctgagtaggtgtcattctattctggggggtggggtggggcaggacagcaagggggaggattgggaagacaatagcaggcatgctggggatgcggtgggctctatggggtaaccacgtgcggacccaacggccgcaggaacccctagtgatggagttggccactccctctctgcgcgctcgctcgctcactgaggccgggcgaccaaaggtcgcccgacgcccgggctttgcccgggcggcctcagtgagcgagcgagcgcgcagctgcctgcaggggcgcctgatgcggtattttctccttacgcatctgtgcggtatttcacaccgcatacgtcaaagcaaccatagtacgcgccctgtagcggcacattaagcgcggcgggtgtggtggttacgcgcagcgtgaccgctacacttgccagcgccttagcgcccgctcctttcgctttcttcccttcctttctcgccacgttcgccggctttccccgtcaagctctaaatcgggggctccctttagggttccgatttagtgctttacggcacctcgaccccaaaaaacttgatttgggtgatggttcacgtagtgggccatcgccctgatagacggtttttcgccctttgacgttggagtccacgttctttaatagtggactcttgttccaaactggaacaacactcaactctatctcgggctattcttttgatttataagggattttgccgatttcggtctattggttaaaaaatgagctgatttaacaaaaatttaacgcgaattttaacaaaatattaacgtttacaattttatggtgcactctcagtacaatctgctctgatgccgcatagttaagccagccccgacacccgccaacacccgctgacgcgccctgacgggcttgtctgctcccggcatccgcttacagacaagctgtgaccgtctccgggagctgcatgtgtcagaggttttcaccgtcatcaccgaaacgcgcgagacgaaagggcctcgtgatacgcctatttttataggttaatgtcatgataataatggtttcttagacgtcaggtggcacttttcggggaaatgtgcgcggaacccctatttgtttatttttctaaatacattcaaatatgtatccgctcatgagacaataaccctgataaatgcttcaataatattgaaaaaggaagagtcctgaggcggaaagaaccagctgtggaatgtgtgtcagttagggtgtggaaagtccccaggctccccagcaggcagaagtatgcaaagcatgcatctcaattagtcagcaaccaggtgtggaaagtccccaggctccccagcaggcagaagtatgcaaagcatgcatctcaattagtcagcaaccatagtcccgcccctaactccgcccatcccgcccctaactccgcccagttccgcccattctccgccccatggctgactaattttttttatttatgcagaggccgaggccgcctcggcctctgagctattccagaagtagtgaggaggcttttttggaggcctaggcttttgcaaagatcgatcaagagacaggatgaggatcgtttcgcatgattgaacaagatggattgcacgcaggttctccggccgcttgggtggagaggctattcggctatgactgggcacaacagacaatcggctgctctgatgccgccgtgttccggctgtcagcgcaggggcgcccggttctttttgtcaagaccgacctgtccggtgccctgaatgaactgcaagacgaggcagcgcggctatcgtggctggccacgacgggcgttccttgcgcagctgtgctcgacgttgtcactgaagcgggaagggactggctgctattgggcgaagtgccggggcaggatctcctgtcatctcaccttgctcctgccgagaaagtatccatcatggctgatgcaatgcggcggctgcatacgcttgatccggctacctgcccattcgaccaccaagcgaaacatcgcatcgagcgagcacgtactcggatggaagccggtcttgtcgatcaggatgatctggacgaagagcatcaggggctcgcgccagccgaactgttcgccaggctcaaggcgagcatgcccgacggcgaggatctcgtcgtgacccatggcgatgcctgcttgccgaatatcatggtggaaaatggccgcttttctggattcatcgactgtggccggctgggtgtggcggaccgctatcaggacatagcgttggctacccgtgatattgctgaagagcttggcggcgaatgggctgaccgcttcctcgtgctttacggtatcgccgctcccgattcgcagcgcatcgccttctatcgccttcttgacgagttcttctgactgtcagaccaagtttactcatatatactttagattgatttaaaacttcatttttaatttaaaaggatctaggtgaagatcctttttgataatctcatgaccaaaatcccttaacgtgagttttcgttccactgagcgtcagaccccgtagaaaagatcaaaggatcttcttgagatcctttttttctgcgcgtaatctgctgcttgcaaacaaaaaaaccaccgctaccagcggtggtttgtttgccggatcaagagctaccaactctttttccgaaggtaactggcttcagcagagcgcagataccaaatactgttcttctagtgtagccgtagttaggccaccacttcaagaactctgtagcaccgcctacatacctcgctctgctaatcctgttaccagtggctgctgccagtggcgataagtcgtgtcttaccgggttggactcaagacgatagttaccggataaggcgcagcggtcgggctgaacggggggttcgtgcacacagcccagcttggagcgaacgacctacaccgaactgagatacctacagcgtgagctatgagaaagcgccacgcttcccgaagggagaaaggcggacaggtatccggtaagcggcagggtcggaacaggagagcgcacgagggagcttccagggggaaacgcctggtatctttatagtcctgtcgggtttcgccacctctgacttgagcgtcgatttttgtgatgctcgtcaggggggcggagcctatggaaaaacgccagcaacgcggcctttttacggttcctggccttttgctggccttttgctcacatgt

SEQ ID NO: 4 - DNA, 4853 bp, 人工序列（Artificial Sequence）
  pAV-CAG-spRS1-RdCVF-BGH
cctgcaggcagctgcgcgctcgctcgctcactgaggccgcccgggcgtcgggcgacctttggtcgcccggcctcagtgagcgagcgagcgcgcagagagggagtggccaactccatcactaggggttcctgcggccggtcgcgtctagtactagtctagtcgcgtaccattgacgtcaataatgacgtatgttcccatagtaacgccaatagggactttccattgacgtcaatgggtggagtatttacggtaaactgcccacttggcagtacatcaagtgtatcatatgccaagtacgccccctattgacgtcaatgacggtaaatggcccgcctggcattatgcccagtacatgaccttatgggactttcctacttggcagtacatctacgtattagtcatcgctattaccatggtcgaggtgagccccacgttctgcttcactctccccatctcccccccctccccacccccaattttgtatttatttattttttaattattttgtgcagcgatgggggcggggggggggggggggcgcgcgccaggcggggcggggcggggcgaggggcggggcggggcgaggcggagaggtgcggcggcagccaatcagagcggcgcgctccgaaagtttccttttatggcgaggcggcggcggcggcggccctataaaaagcgaagcgcgcggcgggcgggagtcgctgcgacgctgccttcgccccgtgccccgctccgccgccgcctcgcgccgcccgccccggctctgactgaccgcgttactcccacaggtgagcgggcgggacggcccttctcctccgggctgtaattagcgcttggtttaatgacggcttgtttcttttctgtggctgcgtgaaagccttgaggggctccgggagggccctttgtgcggggggagcggctcggggctgtccgcggggggacggctgccttcgggggggacggggcagggcggggttcggcttctggcgtgtgaccggcggctctagagcctctgctaaccatgttcatgccttcttctttttcctacagctcctgggcaacgtgctggttattgtgctgtctcatcattttggcaaagaattggatcggtaccgaggagatctgccaccatgagcagaaagatcgagggcttcctgctcctgctcctgttcggctacgaggccaccctgggcctgagcgcctccctgttctctggccgcatcctgatccgcaacaatagcgaccaggacgagctggatacggaggctgaggtcagtcgcaggctggagaaccggctggtgctgctgttctttggtgctggggcttgtccacagtgccaggccttcgtgcccatcctcaaggacttcttcgtgcggctcacagatgagttctatgtactgcgggcggctcagctggccctggtgtacgtgtcccaggactccacggaggagcagcaggacctgttcctcaaggacatgccaaagaaatggcttttcctgccctttgaggatgatctgaggaggtgataaacgcgtctgtgccttctagttgccagccatctgttgtttgcccctcccccgtgccttccttgaccctggaaggtgccactcccactgtcctttcctaataaaatgaggaaattgcatcgcattgtctgagtaggtgtcattctattctggggggtggggtggggcaggacagcaagggggaggattgggaagacaatagcaggcatgctggggatgcggtgggctctatggggtaaccacgtgcggacccaacggccgcaggaacccctagtgatggagttggccactccctctctgcgcgctcgctcgctcactgaggccgggcgaccaaaggtcgcccgacgcccgggctttgcccgggcggcctcagtgagcgagcgagcgcgcagctgcctgcaggggcgcctgatgcggtattttctccttacgcatctgtgcggtatttcacaccgcatacgtcaaagcaaccatagtacgcgccctgtagcggcacattaagcgcggcgggtgtggtggttacgcgcagcgtgaccgctacacttgccagcgccttagcgcccgctcctttcgctttcttcccttcctttctcgccacgttcgccggctttccccgtcaagctctaaatcgggggctccctttagggttccgatttagtgctttacggcacctcgaccccaaaaaacttgatttgggtgatggttcacgtagtgggccatcgccctgatagacggtttttcgccctttgacgttggagtccacgttctttaatagtggactcttgttccaaactggaacaacactcaactctatctcgggctattcttttgatttataagggattttgccgatttcggtctattggttaaaaaatgagctgatttaacaaaaatttaacgcgaattttaacaaaatattaacgtttacaattttatggtgcactctcagtacaatctgctctgatgccgcatagttaagccagccccgacacccgccaacacccgctgacgcgccctgacgggcttgtctgctcccggcatccgcttacagacaagctgtgaccgtctccgggagctgcatgtgtcagaggttttcaccgtcatcaccgaaacgcgcgagacgaaagggcctcgtgatacgcctatttttataggttaatgtcatgataataatggtttcttagacgtcaggtggcacttttcggggaaatgtgcgcggaacccctatttgtttatttttctaaatacattcaaatatgtatccgctcatgagacaataaccctgataaatgcttcaataatattgaaaaaggaagagtcctgaggcggaaagaaccagctgtggaatgtgtgtcagttagggtgtggaaagtccccaggctccccagcaggcagaagtatgcaaagcatgcatctcaattagtcagcaaccaggtgtggaaagtccccaggctccccagcaggcagaagtatgcaaagcatgcatctcaattagtcagcaaccatagtcccgcccctaactccgcccatcccgcccctaactccgcccagttccgcccattctccgccccatggctgactaattttttttatttatgcagaggccgaggccgcctcggcctctgagctattccagaagtagtgaggaggcttttttggaggcctaggcttttgcaaagatcgatcaagagacaggatgaggatcgtttcgcatgattgaacaagatggattgcacgcaggttctccggccgcttgggtggagaggctattcggctatgactgggcacaacagacaatcggctgctctgatgccgccgtgttccggctgtcagcgcaggggcgcccggttctttttgtcaagaccgacctgtccggtgccctgaatgaactgcaagacgaggcagcgcggctatcgtggctggccacgacgggcgttccttgcgcagctgtgctcgacgttgtcactgaagcgggaagggactggctgctattgggcgaagtgccggggcaggatctcctgtcatctcaccttgctcctgccgagaaagtatccatcatggctgatgcaatgcggcggctgcatacgcttgatccggctacctgcccattcgaccaccaagcgaaacatcgcatcgagcgagcacgtactcggatggaagccggtcttgtcgatcaggatgatctggacgaagagcatcaggggctcgcgccagccgaactgttcgccaggctcaaggcgagcatgcccgacggcgaggatctcgtcgtgacccatggcgatgcctgcttgccgaatatcatggtggaaaatggccgcttttctggattcatcgactgtggccggctgggtgtggcggaccgctatcaggacatagcgttggctacccgtgatattgctgaagagcttggcggcgaatgggctgaccgcttcctcgtgctttacggtatcgccgctcccgattcgcagcgcatcgccttctatcgccttcttgacgagttcttctgactgtcagaccaagtttactcatatatactttagattgatttaaaacttcatttttaatttaaaaggatctaggtgaagatcctttttgataatctcatgaccaaaatcccttaacgtgagttttcgttccactgagcgtcagaccccgtagaaaagatcaaaggatcttcttgagatcctttttttctgcgcgtaatctgctgcttgcaaacaaaaaaaccaccgctaccagcggtggtttgtttgccggatcaagagctaccaactctttttccgaaggtaactggcttcagcagagcgcagataccaaatactgttcttctagtgtagccgtagttaggccaccacttcaagaactctgtagcaccgcctacatacctcgctctgctaatcctgttaccagtggctgctgccagtggcgataagtcgtgtcttaccgggttggactcaagacgatagttaccggataaggcgcagcggtcgggctgaacggggggttcgtgcacacagcccagcttggagcgaacgacctacaccgaactgagatacctacagcgtgagctatgagaaagcgccacgcttcccgaagggagaaaggcggacaggtatccggtaagcggcagggtcggaacaggagagcgcacgagggagcttccagggggaaacgcctggtatctttatagtcctgtcgggtttcgccacctctgacttgagcgtcgatttttgtgatgctcgtcaggggggcggagcctatggaaaaacgccagcaacgcggcctttttacggttcctggccttttgctggccttttgctcacatgt

SEQ ID NO: 5 - DNA, 4856 bp, 人工序列（Artificial Sequence）
  pAV-CAG-spNDP-RdCVF-BGH
cctgcaggcagctgcgcgctcgctcgctcactgaggccgcccgggcgtcgggcgacctttggtcgcccggcctcagtgagcgagcgagcgcgcagagagggagtggccaactccatcactaggggttcctgcggccggtcgcgtctagtactagtctagtcgcgtaccattgacgtcaataatgacgtatgttcccatagtaacgccaatagggactttccattgacgtcaatgggtggagtatttacggtaaactgcccacttggcagtacatcaagtgtatcatatgccaagtacgccccctattgacgtcaatgacggtaaatggcccgcctggcattatgcccagtacatgaccttatgggactttcctacttggcagtacatctacgtattagtcatcgctattaccatggtcgaggtgagccccacgttctgcttcactctccccatctcccccccctccccacccccaattttgtatttatttattttttaattattttgtgcagcgatgggggcggggggggggggggggcgcgcgccaggcggggcggggcggggcgaggggcggggcggggcgaggcggagaggtgcggcggcagccaatcagagcggcgcgctccgaaagtttccttttatggcgaggcggcggcggcggcggccctataaaaagcgaagcgcgcggcgggcgggagtcgctgcgacgctgccttcgccccgtgccccgctccgccgccgcctcgcgccgcccgccccggctctgactgaccgcgttactcccacaggtgagcgggcgggacggcccttctcctccgggctgtaattagcgcttggtttaatgacggcttgtttcttttctgtggctgcgtgaaagccttgaggggctccgggagggccctttgtgcggggggagcggctcggggctgtccgcggggggacggctgccttcgggggggacggggcagggcggggttcggcttctggcgtgtgaccggcggctctagagcctctgctaaccatgttcatgccttcttctttttcctacagctcctgggcaacgtgctggttattgtgctgtctcatcattttggcaaagaattggatcggtaccgaggagatctgccaccatgagaaagcacgtgctggccgctagcttcagcatgctgagcctgctggtgatcatgggcgacaccgacagcgcctccctgttctctggccgcatcctgatccgcaacaatagcgaccaggacgagctggatacggaggctgaggtcagtcgcaggctggagaaccggctggtgctgctgttctttggtgctggggcttgtccacagtgccaggccttcgtgcccatcctcaaggacttcttcgtgcggctcacagatgagttctatgtactgcgggcggctcagctggccctggtgtacgtgtcccaggactccacggaggagcagcaggacctgttcctcaaggacatgccaaagaaatggcttttcctgccctttgaggatgatctgaggaggtgataaacgcgtctgtgccttctagttgccagccatctgttgtttgcccctcccccgtgccttccttgaccctggaaggtgccactcccactgtcctttcctaataaaatgaggaaattgcatcgcattgtctgagtaggtgtcattctattctggggggtggggtggggcaggacagcaagggggaggattgggaagacaatagcaggcatgctggggatgcggtgggctctatggggtaaccacgtgcggacccaacggccgcaggaacccctagtgatggagttggccactccctctctgcgcgctcgctcgctcactgaggccgggcgaccaaaggtcgcccgacgcccgggctttgcccgggcggcctcagtgagcgagcgagcgcgcagctgcctgcaggggcgcctgatgcggtattttctccttacgcatctgtgcggtatttcacaccgcatacgtcaaagcaaccatagtacgcgccctgtagcggcacattaagcgcggcgggtgtggtggttacgcgcagcgtgaccgctacacttgccagcgccttagcgcccgctcctttcgctttcttcccttcctttctcgccacgttcgccggctttccccgtcaagctctaaatcgggggctccctttagggttccgatttagtgctttacggcacctcgaccccaaaaaacttgatttgggtgatggttcacgtagtgggccatcgccctgatagacggtttttcgccctttgacgttggagtccacgttctttaatagtggactcttgttccaaactggaacaacactcaactctatctcgggctattcttttgatttataagggattttgccgatttcggtctattggttaaaaaatgagctgatttaacaaaaatttaacgcgaattttaacaaaatattaacgtttacaattttatggtgcactctcagtacaatctgctctgatgccgcatagttaagccagccccgacacccgccaacacccgctgacgcgccctgacgggcttgtctgctcccggcatccgcttacagacaagctgtgaccgtctccgggagctgcatgtgtcagaggttttcaccgtcatcaccgaaacgcgcgagacgaaagggcctcgtgatacgcctatttttataggttaatgtcatgataataatggtttcttagacgtcaggtggcacttttcggggaaatgtgcgcggaacccctatttgtttatttttctaaatacattcaaatatgtatccgctcatgagacaataaccctgataaatgcttcaataatattgaaaaaggaagagtcctgaggcggaaagaaccagctgtggaatgtgtgtcagttagggtgtggaaagtccccaggctccccagcaggcagaagtatgcaaagcatgcatctcaattagtcagcaaccaggtgtggaaagtccccaggctccccagcaggcagaagtatgcaaagcatgcatctcaattagtcagcaaccatagtcccgcccctaactccgcccatcccgcccctaactccgcccagttccgcccattctccgccccatggctgactaattttttttatttatgcagaggccgaggccgcctcggcctctgagctattccagaagtagtgaggaggcttttttggaggcctaggcttttgcaaagatcgatcaagagacaggatgaggatcgtttcgcatgattgaacaagatggattgcacgcaggttctccggccgcttgggtggagaggctattcggctatgactgggcacaacagacaatcggctgctctgatgccgccgtgttccggctgtcagcgcaggggcgcccggttctttttgtcaagaccgacctgtccggtgccctgaatgaactgcaagacgaggcagcgcggctatcgtggctggccacgacgggcgttccttgcgcagctgtgctcgacgttgtcactgaagcgggaagggactggctgctattgggcgaagtgccggggcaggatctcctgtcatctcaccttgctcctgccgagaaagtatccatcatggctgatgcaatgcggcggctgcatacgcttgatccggctacctgcccattcgaccaccaagcgaaacatcgcatcgagcgagcacgtactcggatggaagccggtcttgtcgatcaggatgatctggacgaagagcatcaggggctcgcgccagccgaactgttcgccaggctcaaggcgagcatgcccgacggcgaggatctcgtcgtgacccatggcgatgcctgcttgccgaatatcatggtggaaaatggccgcttttctggattcatcgactgtggccggctgggtgtggcggaccgctatcaggacatagcgttggctacccgtgatattgctgaagagcttggcggcgaatgggctgaccgcttcctcgtgctttacggtatcgccgctcccgattcgcagcgcatcgccttctatcgccttcttgacgagttcttctgactgtcagaccaagtttactcatatatactttagattgatttaaaacttcatttttaatttaaaaggatctaggtgaagatcctttttgataatctcatgaccaaaatcccttaacgtgagttttcgttccactgagcgtcagaccccgtagaaaagatcaaaggatcttcttgagatcctttttttctgcgcgtaatctgctgcttgcaaacaaaaaaaccaccgctaccagcggtggtttgtttgccggatcaagagctaccaactctttttccgaaggtaactggcttcagcagagcgcagataccaaatactgttcttctagtgtagccgtagttaggccaccacttcaagaactctgtagcaccgcctacatacctcgctctgctaatcctgttaccagtggctgctgccagtggcgataagtcgtgtcttaccgggttggactcaagacgatagttaccggataaggcgcagcggtcgggctgaacggggggttcgtgcacacagcccagcttggagcgaacgacctacaccgaactgagatacctacagcgtgagctatgagaaagcgccacgcttcccgaagggagaaaggcggacaggtatccggtaagcggcagggtcggaacaggagagcgcacgagggagcttccagggggaaacgcctggtatctttatagtcctgtcgggtttcgccacctctgacttgagcgtcgatttttgtgatgctcgtcaggggggcggagcctatggaaaaacgccagcaacgcggcctttttacggttcctggccttttgctggccttttgctcacatgt

SEQ ID NO: 6 - DNA, 4874 bp, 人工序列（Artificial Sequence）
  pAV-CAG-spGAS6-RdCVF-BGH
cctgcaggcagctgcgcgctcgctcgctcactgaggccgcccgggcgtcgggcgacctttggtcgcccggcctcagtgagcgagcgagcgcgcagagagggagtggccaactccatcactaggggttcctgcggccggtcgcgtctagtactagtctagtcgcgtaccattgacgtcaataatgacgtatgttcccatagtaacgccaatagggactttccattgacgtcaatgggtggagtatttacggtaaactgcccacttggcagtacatcaagtgtatcatatgccaagtacgccccctattgacgtcaatgacggtaaatggcccgcctggcattatgcccagtacatgaccttatgggactttcctacttggcagtacatctacgtattagtcatcgctattaccatggtcgaggtgagccccacgttctgcttcactctccccatctcccccccctccccacccccaattttgtatttatttattttttaattattttgtgcagcgatgggggcggggggggggggggggcgcgcgccaggcggggcggggcggggcgaggggcggggcggggcgaggcggagaggtgcggcggcagccaatcagagcggcgcgctccgaaagtttccttttatggcgaggcggcggcggcggcggccctataaaaagcgaagcgcgcggcgggcgggagtcgctgcgacgctgccttcgccccgtgccccgctccgccgccgcctcgcgccgcccgccccggctctgactgaccgcgttactcccacaggtgagcgggcgggacggcccttctcctccgggctgtaattagcgcttggtttaatgacggcttgtttcttttctgtggctgcgtgaaagccttgaggggctccgggagggccctttgtgcggggggagcggctcggggctgtccgcggggggacggctgccttcgggggggacggggcagggcggggttcggcttctggcgtgtgaccggcggctctagagcctctgctaaccatgttcatgccttcttctttttcctacagctcctgggcaacgtgctggttattgtgctgtctcatcattttggcaaagaattggatcggtaccgaggagatctgccaccatggccccctccctgagccccggccccgccgccctcagaagagctcctcagctgctcctgctcctgctggccgccgagtgcgccctggccgcctccctgttctctggccgcatcctgatccgcaacaatagcgaccaggacgagctggatacggaggctgaggtcagtcgcaggctggagaaccggctggtgctgctgttctttggtgctggggcttgtccacagtgccaggccttcgtgcccatcctcaaggacttcttcgtgcggctcacagatgagttctatgtactgcgggcggctcagctggccctggtgtacgtgtcccaggactccacggaggagcagcaggacctgttcctcaaggacatgccaaagaaatggcttttcctgccctttgaggatgatctgaggaggtgataaacgcgtctgtgccttctagttgccagccatctgttgtttgcccctcccccgtgccttccttgaccctggaaggtgccactcccactgtcctttcctaataaaatgaggaaattgcatcgcattgtctgagtaggtgtcattctattctggggggtggggtggggcaggacagcaagggggaggattgggaagacaatagcaggcatgctggggatgcggtgggctctatggggtaaccacgtgcggacccaacggccgcaggaacccctagtgatggagttggccactccctctctgcgcgctcgctcgctcactgaggccgggcgaccaaaggtcgcccgacgcccgggctttgcccgggcggcctcagtgagcgagcgagcgcgcagctgcctgcaggggcgcctgatgcggtattttctccttacgcatctgtgcggtatttcacaccgcatacgtcaaagcaaccatagtacgcgccctgtagcggcacattaagcgcggcgggtgtggtggttacgcgcagcgtgaccgctacacttgccagcgccttagcgcccgctcctttcgctttcttcccttcctttctcgccacgttcgccggctttccccgtcaagctctaaatcgggggctccctttagggttccgatttagtgctttacggcacctcgaccccaaaaaacttgatttgggtgatggttcacgtagtgggccatcgccctgatagacggtttttcgccctttgacgttggagtccacgttctttaatagtggactcttgttccaaactggaacaacactcaactctatctcgggctattcttttgatttataagggattttgccgatttcggtctattggttaaaaaatgagctgatttaacaaaaatttaacgcgaattttaacaaaatattaacgtttacaattttatggtgcactctcagtacaatctgctctgatgccgcatagttaagccagccccgacacccgccaacacccgctgacgcgccctgacgggcttgtctgctcccggcatccgcttacagacaagctgtgaccgtctccgggagctgcatgtgtcagaggttttcaccgtcatcaccgaaacgcgcgagacgaaagggcctcgtgatacgcctatttttataggttaatgtcatgataataatggtttcttagacgtcaggtggcacttttcggggaaatgtgcgcggaacccctatttgtttatttttctaaatacattcaaatatgtatccgctcatgagacaataaccctgataaatgcttcaataatattgaaaaaggaagagtcctgaggcggaaagaaccagctgtggaatgtgtgtcagttagggtgtggaaagtccccaggctccccagcaggcagaagtatgcaaagcatgcatctcaattagtcagcaaccaggtgtggaaagtccccaggctccccagcaggcagaagtatgcaaagcatgcatctcaattagtcagcaaccatagtcccgcccctaactccgcccatcccgcccctaactccgcccagttccgcccattctccgccccatggctgactaattttttttatttatgcagaggccgaggccgcctcggcctctgagctattccagaagtagtgaggaggcttttttggaggcctaggcttttgcaaagatcgatcaagagacaggatgaggatcgtttcgcatgattgaacaagatggattgcacgcaggttctccggccgcttgggtggagaggctattcggctatgactgggcacaacagacaatcggctgctctgatgccgccgtgttccggctgtcagcgcaggggcgcccggttctttttgtcaagaccgacctgtccggtgccctgaatgaactgcaagacgaggcagcgcggctatcgtggctggccacgacgggcgttccttgcgcagctgtgctcgacgttgtcactgaagcgggaagggactggctgctattgggcgaagtgccggggcaggatctcctgtcatctcaccttgctcctgccgagaaagtatccatcatggctgatgcaatgcggcggctgcatacgcttgatccggctacctgcccattcgaccaccaagcgaaacatcgcatcgagcgagcacgtactcggatggaagccggtcttgtcgatcaggatgatctggacgaagagcatcaggggctcgcgccagccgaactgttcgccaggctcaaggcgagcatgcccgacggcgaggatctcgtcgtgacccatggcgatgcctgcttgccgaatatcatggtggaaaatggccgcttttctggattcatcgactgtggccggctgggtgtggcggaccgctatcaggacatagcgttggctacccgtgatattgctgaagagcttggcggcgaatgggctgaccgcttcctcgtgctttacggtatcgccgctcccgattcgcagcgcatcgccttctatcgccttcttgacgagttcttctgactgtcagaccaagtttactcatatatactttagattgatttaaaacttcatttttaatttaaaaggatctaggtgaagatcctttttgataatctcatgaccaaaatcccttaacgtgagttttcgttccactgagcgtcagaccccgtagaaaagatcaaaggatcttcttgagatcctttttttctgcgcgtaatctgctgcttgcaaacaaaaaaaccaccgctaccagcggtggtttgtttgccggatcaagagctaccaactctttttccgaaggtaactggcttcagcagagcgcagataccaaatactgttcttctagtgtagccgtagttaggccaccacttcaagaactctgtagcaccgcctacatacctcgctctgctaatcctgttaccagtggctgctgccagtggcgataagtcgtgtcttaccgggttggactcaagacgatagttaccggataaggcgcagcggtcgggctgaacggggggttcgtgcacacagcccagcttggagcgaacgacctacaccgaactgagatacctacagcgtgagctatgagaaagcgccacgcttcccgaagggagaaaggcggacaggtatccggtaagcggcagggtcggaacaggagagcgcacgagggagcttccagggggaaacgcctggtatctttatagtcctgtcgggtttcgccacctctgacttgagcgtcgatttttgtgatgctcgtcaggggggcggagcctatggaaaaacgccagcaacgcggcctttttacggttcctggccttttgctggccttttgctcacatgt

SEQ ID NO: 7 - DNA, 4865 bp, 人工序列（Artificial Sequence）
  pAV-CAG-spCRB1-RdCVF-BGH
cctgcaggcagctgcgcgctcgctcgctcactgaggccgcccgggcgtcgggcgacctttggtcgcccggcctcagtgagcgagcgagcgcgcagagagggagtggccaactccatcactaggggttcctgcggccggtcgcgtctagtactagtctagtcgcgtaccattgacgtcaataatgacgtatgttcccatagtaacgccaatagggactttccattgacgtcaatgggtggagtatttacggtaaactgcccacttggcagtacatcaagtgtatcatatgccaagtacgccccctattgacgtcaatgacggtaaatggcccgcctggcattatgcccagtacatgaccttatgggactttcctacttggcagtacatctacgtattagtcatcgctattaccatggtcgaggtgagccccacgttctgcttcactctccccatctcccccccctccccacccccaattttgtatttatttattttttaattattttgtgcagcgatgggggcggggggggggggggggcgcgcgccaggcggggcggggcggggcgaggggcggggcggggcgaggcggagaggtgcggcggcagccaatcagagcggcgcgctccgaaagtttccttttatggcgaggcggcggcggcggcggccctataaaaagcgaagcgcgcggcgggcgggagtcgctgcgacgctgccttcgccccgtgccccgctccgccgccgcctcgcgccgcccgccccggctctgactgaccgcgttactcccacaggtgagcgggcgggacggcccttctcctccgggctgtaattagcgcttggtttaatgacggcttgtttcttttctgtggctgcgtgaaagccttgaggggctccgggagggccctttgtgcggggggagcggctcggggctgtccgcggggggacggctgccttcgggggggacggggcagggcggggttcggcttctggcgtgtgaccggcggctctagagcctctgctaaccatgttcatgccttcttctttttcctacagctcctgggcaacgtgctggttattgtgctgtctcatcattttggcaaagaattggatcggtaccgaggagatctgccaccatggccctgaagaacatcaactacctgctgatcttctacctgagcttcagcctgctgatctacatcaagaacagcttctgcgcctccctgttctctggccgcatcctgatccgcaacaatagcgaccaggacgagctggatacggaggctgaggtcagtcgcaggctggagaaccggctggtgctgctgttctttggtgctggggcttgtccacagtgccaggccttcgtgcccatcctcaaggacttcttcgtgcggctcacagatgagttctatgtactgcgggcggctcagctggccctggtgtacgtgtcccaggactccacggaggagcagcaggacctgttcctcaaggacatgccaaagaaatggcttttcctgccctttgaggatgatctgaggaggtgataaacgcgtctgtgccttctagttgccagccatctgttgtttgcccctcccccgtgccttccttgaccctggaaggtgccactcccactgtcctttcctaataaaatgaggaaattgcatcgcattgtctgagtaggtgtcattctattctggggggtggggtggggcaggacagcaagggggaggattgggaagacaatagcaggcatgctggggatgcggtgggctctatggggtaaccacgtgcggacccaacggccgcaggaacccctagtgatggagttggccactccctctctgcgcgctcgctcgctcactgaggccgggcgaccaaaggtcgcccgacgcccgggctttgcccgggcggcctcagtgagcgagcgagcgcgcagctgcctgcaggggcgcctgatgcggtattttctccttacgcatctgtgcggtatttcacaccgcatacgtcaaagcaaccatagtacgcgccctgtagcggcacattaagcgcggcgggtgtggtggttacgcgcagcgtgaccgctacacttgccagcgccttagcgcccgctcctttcgctttcttcccttcctttctcgccacgttcgccggctttccccgtcaagctctaaatcgggggctccctttagggttccgatttagtgctttacggcacctcgaccccaaaaaacttgatttgggtgatggttcacgtagtgggccatcgccctgatagacggtttttcgccctttgacgttggagtccacgttctttaatagtggactcttgttccaaactggaacaacactcaactctatctcgggctattcttttgatttataagggattttgccgatttcggtctattggttaaaaaatgagctgatttaacaaaaatttaacgcgaattttaacaaaatattaacgtttacaattttatggtgcactctcagtacaatctgctctgatgccgcatagttaagccagccccgacacccgccaacacccgctgacgcgccctgacgggcttgtctgctcccggcatccgcttacagacaagctgtgaccgtctccgggagctgcatgtgtcagaggttttcaccgtcatcaccgaaacgcgcgagacgaaagggcctcgtgatacgcctatttttataggttaatgtcatgataataatggtttcttagacgtcaggtggcacttttcggggaaatgtgcgcggaacccctatttgtttatttttctaaatacattcaaatatgtatccgctcatgagacaataaccctgataaatgcttcaataatattgaaaaaggaagagtcctgaggcggaaagaaccagctgtggaatgtgtgtcagttagggtgtggaaagtccccaggctccccagcaggcagaagtatgcaaagcatgcatctcaattagtcagcaaccaggtgtggaaagtccccaggctccccagcaggcagaagtatgcaaagcatgcatctcaattagtcagcaaccatagtcccgcccctaactccgcccatcccgcccctaactccgcccagttccgcccattctccgccccatggctgactaattttttttatttatgcagaggccgaggccgcctcggcctctgagctattccagaagtagtgaggaggcttttttggaggcctaggcttttgcaaagatcgatcaagagacaggatgaggatcgtttcgcatgattgaacaagatggattgcacgcaggttctccggccgcttgggtggagaggctattcggctatgactgggcacaacagacaatcggctgctctgatgccgccgtgttccggctgtcagcgcaggggcgcccggttctttttgtcaagaccgacctgtccggtgccctgaatgaactgcaagacgaggcagcgcggctatcgtggctggccacgacgggcgttccttgcgcagctgtgctcgacgttgtcactgaagcgggaagggactggctgctattgggcgaagtgccggggcaggatctcctgtcatctcaccttgctcctgccgagaaagtatccatcatggctgatgcaatgcggcggctgcatacgcttgatccggctacctgcccattcgaccaccaagcgaaacatcgcatcgagcgagcacgtactcggatggaagccggtcttgtcgatcaggatgatctggacgaagagcatcaggggctcgcgccagccgaactgttcgccaggctcaaggcgagcatgcccgacggcgaggatctcgtcgtgacccatggcgatgcctgcttgccgaatatcatggtggaaaatggccgcttttctggattcatcgactgtggccggctgggtgtggcggaccgctatcaggacatagcgttggctacccgtgatattgctgaagagcttggcggcgaatgggctgaccgcttcctcgtgctttacggtatcgccgctcccgattcgcagcgcatcgccttctatcgccttcttgacgagttcttctgactgtcagaccaagtttactcatatatactttagattgatttaaaacttcatttttaatttaaaaggatctaggtgaagatcctttttgataatctcatgaccaaaatcccttaacgtgagttttcgttccactgagcgtcagaccccgtagaaaagatcaaaggatcttcttgagatcctttttttctgcgcgtaatctgctgcttgcaaacaaaaaaaccaccgctaccagcggtggtttgtttgccggatcaagagctaccaactctttttccgaaggtaactggcttcagcagagcgcagataccaaatactgttcttctagtgtagccgtagttaggccaccacttcaagaactctgtagcaccgcctacatacctcgctctgctaatcctgttaccagtggctgctgccagtggcgataagtcgtgtcttaccgggttggactcaagacgatagttaccggataaggcgcagcggtcgggctgaacggggggttcgtgcacacagcccagcttggagcgaacgacctacaccgaactgagatacctacagcgtgagctatgagaaagcgccacgcttcccgaagggagaaaggcggacaggtatccggtaagcggcagggtcggaacaggagagcgcacgagggagcttccagggggaaacgcctggtatctttatagtcctgtcgggtttcgccacctctgacttgagcgtcgatttttgtgatgctcgtcaggggggcggagcctatggaaaaacgccagcaacgcggcctttttacggttcctggccttttgctggccttttgctcacatgt

SEQ ID NO: 8 - DNA, 4868 bp, 人工序列（Artificial Sequence）
  pAV-CAG-spCRB2-RdCVF-BGH
cctgcaggcagctgcgcgctcgctcgctcactgaggccgcccgggcgtcgggcgacctttggtcgcccggcctcagtgagcgagcgagcgcgcagagagggagtggccaactccatcactaggggttcctgcggccggtcgcgtctagtactagtctagtcgcgtaccattgacgtcaataatgacgtatgttcccatagtaacgccaatagggactttccattgacgtcaatgggtggagtatttacggtaaactgcccacttggcagtacatcaagtgtatcatatgccaagtacgccccctattgacgtcaatgacggtaaatggcccgcctggcattatgcccagtacatgaccttatgggactttcctacttggcagtacatctacgtattagtcatcgctattaccatggtcgaggtgagccccacgttctgcttcactctccccatctcccccccctccccacccccaattttgtatttatttattttttaattattttgtgcagcgatgggggcggggggggggggggggcgcgcgccaggcggggcggggcggggcgaggggcggggcggggcgaggcggagaggtgcggcggcagccaatcagagcggcgcgctccgaaagtttccttttatggcgaggcggcggcggcggcggccctataaaaagcgaagcgcgcggcgggcgggagtcgctgcgacgctgccttcgccccgtgccccgctccgccgccgcctcgcgccgcccgccccggctctgactgaccgcgttactcccacaggtgagcgggcgggacggcccttctcctccgggctgtaattagcgcttggtttaatgacggcttgtttcttttctgtggctgcgtgaaagccttgaggggctccgggagggccctttgtgcggggggagcggctcggggctgtccgcggggggacggctgccttcgggggggacggggcagggcggggttcggcttctggcgtgtgaccggcggctctagagcctctgctaaccatgttcatgccttcttctttttcctacagctcctgggcaacgtgctggttattgtgctgtctcatcattttggcaaagaattggatcggtaccgaggagatctgccaccatggccctggctagacctggcacccccgacccccaagccctcgctagcgtcctgctcctgctcctgtgggcccccgccctgagcgcctccctgttctctggccgcatcctgatccgcaacaatagcgaccaggacgagctggatacggaggctgaggtcagtcgcaggctggagaaccggctggtgctgctgttctttggtgctggggcttgtccacagtgccaggccttcgtgcccatcctcaaggacttcttcgtgcggctcacagatgagttctatgtactgcgggcggctcagctggccctggtgtacgtgtcccaggactccacggaggagcagcaggacctgttcctcaaggacatgccaaagaaatggcttttcctgccctttgaggatgatctgaggaggtgataaacgcgtctgtgccttctagttgccagccatctgttgtttgcccctcccccgtgccttccttgaccctggaaggtgccactcccactgtcctttcctaataaaatgaggaaattgcatcgcattgtctgagtaggtgtcattctattctggggggtggggtggggcaggacagcaagggggaggattgggaagacaatagcaggcatgctggggatgcggtgggctctatggggtaaccacgtgcggacccaacggccgcaggaacccctagtgatggagttggccactccctctctgcgcgctcgctcgctcactgaggccgggcgaccaaaggtcgcccgacgcccgggctttgcccgggcggcctcagtgagcgagcgagcgcgcagctgcctgcaggggcgcctgatgcggtattttctccttacgcatctgtgcggtatttcacaccgcatacgtcaaagcaaccatagtacgcgccctgtagcggcacattaagcgcggcgggtgtggtggttacgcgcagcgtgaccgctacacttgccagcgccttagcgcccgctcctttcgctttcttcccttcctttctcgccacgttcgccggctttccccgtcaagctctaaatcgggggctccctttagggttccgatttagtgctttacggcacctcgaccccaaaaaacttgatttgggtgatggttcacgtagtgggccatcgccctgatagacggtttttcgccctttgacgttggagtccacgttctttaatagtggactcttgttccaaactggaacaacactcaactctatctcgggctattcttttgatttataagggattttgccgatttcggtctattggttaaaaaatgagctgatttaacaaaaatttaacgcgaattttaacaaaatattaacgtttacaattttatggtgcactctcagtacaatctgctctgatgccgcatagttaagccagccccgacacccgccaacacccgctgacgcgccctgacgggcttgtctgctcccggcatccgcttacagacaagctgtgaccgtctccgggagctgcatgtgtcagaggttttcaccgtcatcaccgaaacgcgcgagacgaaagggcctcgtgatacgcctatttttataggttaatgtcatgataataatggtttcttagacgtcaggtggcacttttcggggaaatgtgcgcggaacccctatttgtttatttttctaaatacattcaaatatgtatccgctcatgagacaataaccctgataaatgcttcaataatattgaaaaaggaagagtcctgaggcggaaagaaccagctgtggaatgtgtgtcagttagggtgtggaaagtccccaggctccccagcaggcagaagtatgcaaagcatgcatctcaattagtcagcaaccaggtgtggaaagtccccaggctccccagcaggcagaagtatgcaaagcatgcatctcaattagtcagcaaccatagtcccgcccctaactccgcccatcccgcccctaactccgcccagttccgcccattctccgccccatggctgactaattttttttatttatgcagaggccgaggccgcctcggcctctgagctattccagaagtagtgaggaggcttttttggaggcctaggcttttgcaaagatcgatcaagagacaggatgaggatcgtttcgcatgattgaacaagatggattgcacgcaggttctccggccgcttgggtggagaggctattcggctatgactgggcacaacagacaatcggctgctctgatgccgccgtgttccggctgtcagcgcaggggcgcccggttctttttgtcaagaccgacctgtccggtgccctgaatgaactgcaagacgaggcagcgcggctatcgtggctggccacgacgggcgttccttgcgcagctgtgctcgacgttgtcactgaagcgggaagggactggctgctattgggcgaagtgccggggcaggatctcctgtcatctcaccttgctcctgccgagaaagtatccatcatggctgatgcaatgcggcggctgcatacgcttgatccggctacctgcccattcgaccaccaagcgaaacatcgcatcgagcgagcacgtactcggatggaagccggtcttgtcgatcaggatgatctggacgaagagcatcaggggctcgcgccagccgaactgttcgccaggctcaaggcgagcatgcccgacggcgaggatctcgtcgtgacccatggcgatgcctgcttgccgaatatcatggtggaaaatggccgcttttctggattcatcgactgtggccggctgggtgtggcggaccgctatcaggacatagcgttggctacccgtgatattgctgaagagcttggcggcgaatgggctgaccgcttcctcgtgctttacggtatcgccgctcccgattcgcagcgcatcgccttctatcgccttcttgacgagttcttctgactgtcagaccaagtttactcatatatactttagattgatttaaaacttcatttttaatttaaaaggatctaggtgaagatcctttttgataatctcatgaccaaaatcccttaacgtgagttttcgttccactgagcgtcagaccccgtagaaaagatcaaaggatcttcttgagatcctttttttctgcgcgtaatctgctgcttgcaaacaaaaaaaccaccgctaccagcggtggtttgtttgccggatcaagagctaccaactctttttccgaaggtaactggcttcagcagagcgcagataccaaatactgttcttctagtgtagccgtagttaggccaccacttcaagaactctgtagcaccgcctacatacctcgctctgctaatcctgttaccagtggctgctgccagtggcgataagtcgtgtcttaccgggttggactcaagacgatagttaccggataaggcgcagcggtcgggctgaacggggggttcgtgcacacagcccagcttggagcgaacgacctacaccgaactgagatacctacagcgtgagctatgagaaagcgccacgcttcccgaagggagaaaggcggacaggtatccggtaagcggcagggtcggaacaggagagcgcacgagggagcttccagggggaaacgcctggtatctttatagtcctgtcgggtttcgccacctctgacttgagcgtcgatttttgtgatgctcgtcaggggggcggagcctatggaaaaacgccagcaacgcggcctttttacggttcctggccttttgctggccttttgctcacatgt

SEQ ID NO: 9 - DNA, 7728 bp, 人工序列（Artificial Sequence）
  pAV-CAG-CYP4V2-BGH-CAG-RdCVF-BGH
cctgcaggcagctgcgcgctcgctcgctcactgaggccgcccgggcgtcgggcgacctttggtcgcccggcctcagtgagcgagcgagcgcgcagagagggagtggccaactccatcactaggggttcctgcggccggtcgcgtctagtactagtctagtcgcgtaccattgacgtcaataatgacgtatgttcccatagtaacgccaatagggactttccattgacgtcaatgggtggagtatttacggtaaactgcccacttggcagtacatcaagtgtatcatatgccaagtacgccccctattgacgtcaatgacggtaaatggcccgcctggcattatgcccagtacatgaccttatgggactttcctacttggcagtacatctacgtattagtcatcgctattaccatggtcgaggtgagccccacgttctgcttcactctccccatctcccccccctccccacccccaattttgtatttatttattttttaattattttgtgcagcgatgggggcggggggggggggggggcgcgcgccaggcggggcggggcggggcgaggggcggggcggggcgaggcggagaggtgcggcggcagccaatcagagcggcgcgctccgaaagtttccttttatggcgaggcggcggcggcggcggccctataaaaagcgaagcgcgcggcgggcgggagtcgctgcgacgctgccttcgccccgtgccccgctccgccgccgcctcgcgccgcccgccccggctctgactgaccgcgttactcccacaggtgagcgggcgggacggcccttctcctccgggctgtaattagcgcttggtttaatgacggcttgtttcttttctgtggctgcgtgaaagccttgaggggctccgggagggccctttgtgcggggggagcggctcggggctgtccgcggggggacggctgccttcgggggggacggggcagggcggggttcggcttctggcgtgtgaccggcggctctagagcctctgctaaccatgttcatgccttcttctttttcctacagctcctgggcaacgtgctggttattgtgctgtctcatcattttggcaaagaattggatcggtaccgaggagatctgccaccatggcggggctctggctggggctcgtgtggcagaagctgctgctgtggggcgcggcgagtgccctttccctggccggcgccagtctggtcctgagtctgctgcagagggtggcgagctacgcgcggaaatggcagcagatgcggcccatccccacggtggcccgcgcctacccactggtgggccacgcgctgctgatgaagccggacgggcgagaattttttcagcagatcattgagtacacagaggaataccgccacatgccgctgctgaagctctgggtcgggccagtgcccatggtggccctttataatgcagaaaatgtggaggtaattttaactagttcaaagcaaattgacaaatcctctatgtacaagtttttagaaccatggcttggcctaggacttcttacaagtactggaaacaaatggcgctccaggagaaagatgttaacacccactttccattttaccattctggaagatttcttagatatcatgaatgaacaagcaaatatattggttaagaaacttgaaaaacacattaaccaagaagcatttaactgctttttttacatcactctttgtgccttagatatcatctgtgaaacagctatggggaagaatattggtgctcaaagtaatgatgattccgagtatgtccgtgcagtttatagaatgagtgagatgatatttcgaagaataaagatgccctggctttggcttgatctctggtaccttatgtttaaagaaggatgggaacacaaaaagagccttcagatcctacatacttttaccaacagtgtcatcgcggaacgggccaatgaaatgaacgccaatgaagactgtagaggtgatggcaggggctctgccccctccaaaaataaacgcagggcctttcttgacttgcttttaagtgtgactgatgacgaagggaacaggctaagtcatgaagatattcgagaagaagttgacaccttcatgtttgaggggcacgatacaactgcagctgcaataaactggtccttatacctgttgggttctaacccagaagtccagaaaaaagtggatcatgaattggatgacgtgtttgggaagtctgaccgtcccgctacagtagaagacctgaagaaacttcggtatctggaatgtgttattaaggagacccttcgcctttttccttctgttcctttatttgcccgtagtgttagtgaagattgtgaagtggcaggttacagagttctaaaaggcactgaagccgtcatcattccctatgcattgcacagagatccgagatacttccccaaccccgaggagttccagcctgagcggttcttccccgagaatgcacaagggcgccatccatatgcctacgtgcccttctctgctggccccaggaactgtataggtcaaaagtttgctgtgatggaagaaaagaccattctttcgtgcatcctgaggcacttttggatagaatccaaccagaaaagagaagagcttggtctagaaggacagttgattcttcgtccaagtaatggcatctggatcaagttgaagaggagaaatgcagatgaacgctaaacgcgtggtttatccgatccaccggatctagataagatatccgatccaccggatctagataactgatcataatcagccataccacatttgtagaggttttacttgctttaaaaaacctcccacacctccccctgaacctgaaacataaaatgaatgcaattggcggccgcctcgagctgtgccttctagttgccagccatctgttgtttgcccctcccccgtgccttccttgaccctggaaggtgccactcccactgtcctttcctaataaaatgaggaaattgcatcgcattgtctgagtaggtgtcattctattctggggggtggggtggggcaggacagcaagggggaggattgggaagacaatagcaggcatgctggggatgcggtgggctctatggggtaaccccattgacgtcaataatgacgtatgttcccatagtaacgccaatagggactttccattgacgtcaatgggtggagtatttacggtaaactgcccacttggcagtacatcaagtgtatcatatgccaagtacgccccctattgacgtcaatgacggtaaatggcccgcctggcattatgcccagtacatgaccttatgggactttcctacttggcagtacatctacgtattagtcatcgctattaccatggtcgaggtgagccccacgttctgcttcactctccccatctcccccccctccccacccccaattttgtatttatttattttttaattattttgtgcagcgatgggggcggggggggggggggggcgcgcgccaggcggggcggggcggggcgaggggcggggcggggcgaggcggagaggtgcggcggcagccaatcagagcggcgcgctccgaaagtttccttttatggcgaggcggcggcggcggcggccctataaaaagcgaagcgcgcggcgggcgggagtcgctgcgacgctgccttcgccccgtgccccgctccgccgccgcctcgcgccgcccgccccggctctgactgaccgcgttactcccacaggtgagcgggcgggacggcccttctcctccgggctgtaattagcgcttggtttaatgacggcttgtttcttttctgtggctgcgtgaaagccttgaggggctccgggagggccctttgtgcggggggagcggctcggggctgtccgcggggggacggctgccttcgggggggacggggcagggcggggttcggcttctggcgtgtgaccggcggctctagagcctctgctaaccatgttcatgccttcttctttttcctacagctcctgggcaacgtgctggttattgtgctgtctcatcattttggcaaagaattggatcggtaccgaggagatctgccaccatggcctccctgttctctggccgcatcctgatccgcaacaatagcgaccaggacgagctggatacggaggctgaggtcagtcgcaggctggagaaccggctggtgctgctgttctttggtgctggggcttgtccacagtgccaggccttcgtgcccatcctcaaggacttcttcgtgcggctcacagatgagttctatgtactgcgggcggctcagctggccctggtgtacgtgtcccaggactccacggaggagcagcaggacctgttcctcaaggacatgccaaagaaatggcttttcctgccctttgaggatgatctgaggaggtgactgtgccttctagttgccagccatctgttgtttgcccctcccccgtgccttccttgaccctggaaggtgccactcccactgtcctttcctaataaaatgaggaaattgcatcgcattgtctgagtaggtgtcattctattctggggggtggggtggggcaggacagcaagggggaggattgggaagacaatagcaggcatgctggggatgcggtgggctctatggggtaaccacgtgcggacccaacggccgcaggaacccctagtgatggagttggccactccctctctgcgcgctcgctcgctcactgaggccgggcgaccaaaggtcgcccgacgcccgggctttgcccgggcggcctcagtgagcgagcgagcgcgcagctgcctgcaggggcgcctgatgcggtattttctccttacgcatctgtgcggtatttcacaccgcatacgtcaaagcaaccatagtacgcgccctgtagcggcacattaagcgcggcgggtgtggtggttacgcgcagcgtgaccgctacacttgccagcgccttagcgcccgctcctttcgctttcttcccttcctttctcgccacgttcgccggctttccccgtcaagctctaaatcgggggctccctttagggttccgatttagtgctttacggcacctcgaccccaaaaaacttgatttgggtgatggttcacgtagtgggccatcgccctgatagacggtttttcgccctttgacgttggagtccacgttctttaatagtggactcttgttccaaactggaacaacactcaactctatctcgggctattcttttgatttataagggattttgccgatttcggtctattggttaaaaaatgagctgatttaacaaaaatttaacgcgaattttaacaaaatattaacgtttacaattttatggtgcactctcagtacaatctgctctgatgccgcatagttaagccagccccgacacccgccaacacccgctgacgcgccctgacgggcttgtctgctcccggcatccgcttacagacaagctgtgaccgtctccgggagctgcatgtgtcagaggttttcaccgtcatcaccgaaacgcgcgagacgaaagggcctcgtgatacgcctatttttataggttaatgtcatgataataatggtttcttagacgtcaggtggcacttttcggggaaatgtgcgcggaacccctatttgtttatttttctaaatacattcaaatatgtatccgctcatgagacaataaccctgataaatgcttcaataatattgaaaaaggaagagtcctgaggcggaaagaaccagctgtggaatgtgtgtcagttagggtgtggaaagtccccaggctccccagcaggcagaagtatgcaaagcatgcatctcaattagtcagcaaccaggtgtggaaagtccccaggctccccagcaggcagaagtatgcaaagcatgcatctcaattagtcagcaaccatagtcccgcccctaactccgcccatcccgcccctaactccgcccagttccgcccattctccgccccatggctgactaattttttttatttatgcagaggccgaggccgcctcggcctctgagctattccagaagtagtgaggaggcttttttggaggcctaggcttttgcaaagatcgatcaagagacaggatgaggatcgtttcgcatgattgaacaagatggattgcacgcaggttctccggccgcttgggtggagaggctattcggctatgactgggcacaacagacaatcggctgctctgatgccgccgtgttccggctgtcagcgcaggggcgcccggttctttttgtcaagaccgacctgtccggtgccctgaatgaactgcaagacgaggcagcgcggctatcgtggctggccacgacgggcgttccttgcgcagctgtgctcgacgttgtcactgaagcgggaagggactggctgctattgggcgaagtgccggggcaggatctcctgtcatctcaccttgctcctgccgagaaagtatccatcatggctgatgcaatgcggcggctgcatacgcttgatccggctacctgcccattcgaccaccaagcgaaacatcgcatcgagcgagcacgtactcggatggaagccggtcttgtcgatcaggatgatctggacgaagagcatcaggggctcgcgccagccgaactgttcgccaggctcaaggcgagcatgcccgacggcgaggatctcgtcgtgacccatggcgatgcctgcttgccgaatatcatggtggaaaatggccgcttttctggattcatcgactgtggccggctgggtgtggcggaccgctatcaggacatagcgttggctacccgtgatattgctgaagagcttggcggcgaatgggctgaccgcttcctcgtgctttacggtatcgccgctcccgattcgcagcgcatcgccttctatcgccttcttgacgagttcttctgactgtcagaccaagtttactcatatatactttagattgatttaaaacttcatttttaatttaaaaggatctaggtgaagatcctttttgataatctcatgaccaaaatcccttaacgtgagttttcgttccactgagcgtcagaccccgtagaaaagatcaaaggatcttcttgagatcctttttttctgcgcgtaatctgctgcttgcaaacaaaaaaaccaccgctaccagcggtggtttgtttgccggatcaagagctaccaactctttttccgaaggtaactggcttcagcagagcgcagataccaaatactgttcttctagtgtagccgtagttaggccaccacttcaagaactctgtagcaccgcctacatacctcgctctgctaatcctgttaccagtggctgctgccagtggcgataagtcgtgtcttaccgggttggactcaagacgatagttaccggataaggcgcagcggtcgggctgaacggggggttcgtgcacacagcccagcttggagcgaacgacctacaccgaactgagatacctacagcgtgagctatgagaaagcgccacgcttcccgaagggagaaaggcggacaggtatccggtaagcggcagggtcggaacaggagagcgcacgagggagcttccagggggaaacgcctggtatctttatagtcctgtcgggtttcgccacctctgacttgagcgtcgatttttgtgatgctcgtcaggggggcggagcctatggaaaaacgccagcaacgcggcctttttacggttcctggccttttgctggccttttgctcacatgt

SEQ ID NO: 10 - DNA, 7776 bp, 人工序列（Artificial Sequence）
  pAV-CAG-CYP4V2-BGH-CAG-spGL-RdCVF-BGH
cctgcaggcagctgcgcgctcgctcgctcactgaggccgcccgggcgtcgggcgacctttggtcgcccggcctcagtgagcgagcgagcgcgcagagagggagtggccaactccatcactaggggttcctgcggccggtcgcgtctagtactagtctagtcgcgtaccattgacgtcaataatgacgtatgttcccatagtaacgccaatagggactttccattgacgtcaatgggtggagtatttacggtaaactgcccacttggcagtacatcaagtgtatcatatgccaagtacgccccctattgacgtcaatgacggtaaatggcccgcctggcattatgcccagtacatgaccttatgggactttcctacttggcagtacatctacgtattagtcatcgctattaccatggtcgaggtgagccccacgttctgcttcactctccccatctcccccccctccccacccccaattttgtatttatttattttttaattattttgtgcagcgatgggggcggggggggggggggggcgcgcgccaggcggggcggggcggggcgaggggcggggcggggcgaggcggagaggtgcggcggcagccaatcagagcggcgcgctccgaaagtttccttttatggcgaggcggcggcggcggcggccctataaaaagcgaagcgcgcggcgggcgggagtcgctgcgacgctgccttcgccccgtgccccgctccgccgccgcctcgcgccgcccgccccggctctgactgaccgcgttactcccacaggtgagcgggcgggacggcccttctcctccgggctgtaattagcgcttggtttaatgacggcttgtttcttttctgtggctgcgtgaaagccttgaggggctccgggagggccctttgtgcggggggagcggctcggggctgtccgcggggggacggctgccttcgggggggacggggcagggcggggttcggcttctggcgtgtgaccggcggctctagagcctctgctaaccatgttcatgccttcttctttttcctacagctcctgggcaacgtgctggttattgtgctgtctcatcattttggcaaagaattggatcggtaccgaggagatctgccaccatggcggggctctggctggggctcgtgtggcagaagctgctgctgtggggcgcggcgagtgccctttccctggccggcgccagtctggtcctgagtctgctgcagagggtggcgagctacgcgcggaaatggcagcagatgcggcccatccccacggtggcccgcgcctacccactggtgggccacgcgctgctgatgaagccggacgggcgagaattttttcagcagatcattgagtacacagaggaataccgccacatgccgctgctgaagctctgggtcgggccagtgcccatggtggccctttataatgcagaaaatgtggaggtaattttaactagttcaaagcaaattgacaaatcctctatgtacaagtttttagaaccatggcttggcctaggacttcttacaagtactggaaacaaatggcgctccaggagaaagatgttaacacccactttccattttaccattctggaagatttcttagatatcatgaatgaacaagcaaatatattggttaagaaacttgaaaaacacattaaccaagaagcatttaactgctttttttacatcactctttgtgccttagatatcatctgtgaaacagctatggggaagaatattggtgctcaaagtaatgatgattccgagtatgtccgtgcagtttatagaatgagtgagatgatatttcgaagaataaagatgccctggctttggcttgatctctggtaccttatgtttaaagaaggatgggaacacaaaaagagccttcagatcctacatacttttaccaacagtgtcatcgcggaacgggccaatgaaatgaacgccaatgaagactgtagaggtgatggcaggggctctgccccctccaaaaataaacgcagggcctttcttgacttgcttttaagtgtgactgatgacgaagggaacaggctaagtcatgaagatattcgagaagaagttgacaccttcatgtttgaggggcacgatacaactgcagctgcaataaactggtccttatacctgttgggttctaacccagaagtccagaaaaaagtggatcatgaattggatgacgtgtttgggaagtctgaccgtcccgctacagtagaagacctgaagaaacttcggtatctggaatgtgttattaaggagacccttcgcctttttccttctgttcctttatttgcccgtagtgttagtgaagattgtgaagtggcaggttacagagttctaaaaggcactgaagccgtcatcattccctatgcattgcacagagatccgagatacttccccaaccccgaggagttccagcctgagcggttcttccccgagaatgcacaagggcgccatccatatgcctacgtgcccttctctgctggccccaggaactgtataggtcaaaagtttgctgtgatggaagaaaagaccattctttcgtgcatcctgaggcacttttggatagaatccaaccagaaaagagaagagcttggtctagaaggacagttgattcttcgtccaagtaatggcatctggatcaagttgaagaggagaaatgcagatgaacgctaaacgcgtggtttatccgatccaccggatctagataagatatccgatccaccggatctagataactgatcataatcagccataccacatttgtagaggttttacttgctttaaaaaacctcccacacctccccctgaacctgaaacataaaatgaatgcaattggcggccgcctcgagctgtgccttctagttgccagccatctgttgtttgcccctcccccgtgccttccttgaccctggaaggtgccactcccactgtcctttcctaataaaatgaggaaattgcatcgcattgtctgagtaggtgtcattctattctggggggtggggtggggcaggacagcaagggggaggattgggaagacaatagcaggcatgctggggatgcggtgggctctatggggtaaccccattgacgtcaataatgacgtatgttcccatagtaacgccaatagggactttccattgacgtcaatgggtggagtatttacggtaaactgcccacttggcagtacatcaagtgtatcatatgccaagtacgccccctattgacgtcaatgacggtaaatggcccgcctggcattatgcccagtacatgaccttatgggactttcctacttggcagtacatctacgtattagtcatcgctattaccatggtcgaggtgagccccacgttctgcttcactctccccatctcccccccctccccacccccaattttgtatttatttattttttaattattttgtgcagcgatgggggcggggggggggggggggcgcgcgccaggcggggcggggcggggcgaggggcggggcggggcgaggcggagaggtgcggcggcagccaatcagagcggcgcgctccgaaagtttccttttatggcgaggcggcggcggcggcggccctataaaaagcgaagcgcgcggcgggcgggagtcgctgcgacgctgccttcgccccgtgccccgctccgccgccgcctcgcgccgcccgccccggctctgactgaccgcgttactcccacaggtgagcgggcgggacggcccttctcctccgggctgtaattagcgcttggtttaatgacggcttgtttcttttctgtggctgcgtgaaagccttgaggggctccgggagggccctttgtgcggggggagcggctcggggctgtccgcggggggacggctgccttcgggggggacggggcagggcggggttcggcttctggcgtgtgaccggcggctctagagcctctgctaaccatgttcatgccttcttctttttcctacagctcctgggcaacgtgctggttattgtgctgtctcatcattttggcaaagaattggatcggtaccgaggagatctgccaccatgggagtcaaagttctgtttgccctgatctgcatcgctgtggccgaggccgcctccctgttctctggccgcatcctgatccgcaacaatagcgaccaggacgagctggatacggaggctgaggtcagtcgcaggctggagaaccggctggtgctgctgttctttggtgctggggcttgtccacagtgccaggccttcgtgcccatcctcaaggacttcttcgtgcggctcacagatgagttctatgtactgcgggcggctcagctggccctggtgtacgtgtcccaggactccacggaggagcagcaggacctgttcctcaaggacatgccaaagaaatggcttttcctgccctttgaggatgatctgaggaggtgactgtgccttctagttgccagccatctgttgtttgcccctcccccgtgccttccttgaccctggaaggtgccactcccactgtcctttcctaataaaatgaggaaattgcatcgcattgtctgagtaggtgtcattctattctggggggtggggtggggcaggacagcaagggggaggattgggaagacaatagcaggcatgctggggatgcggtgggctctatggggtaaccacgtgcggacccaacggccgcaggaacccctagtgatggagttggccactccctctctgcgcgctcgctcgctcactgaggccgggcgaccaaaggtcgcccgacgcccgggctttgcccgggcggcctcagtgagcgagcgagcgcgcagctgcctgcaggggcgcctgatgcggtattttctccttacgcatctgtgcggtatttcacaccgcatacgtcaaagcaaccatagtacgcgccctgtagcggcacattaagcgcggcgggtgtggtggttacgcgcagcgtgaccgctacacttgccagcgccttagcgcccgctcctttcgctttcttcccttcctttctcgccacgttcgccggctttccccgtcaagctctaaatcgggggctccctttagggttccgatttagtgctttacggcacctcgaccccaaaaaacttgatttgggtgatggttcacgtagtgggccatcgccctgatagacggtttttcgccctttgacgttggagtccacgttctttaatagtggactcttgttccaaactggaacaacactcaactctatctcgggctattcttttgatttataagggattttgccgatttcggtctattggttaaaaaatgagctgatttaacaaaaatttaacgcgaattttaacaaaatattaacgtttacaattttatggtgcactctcagtacaatctgctctgatgccgcatagttaagccagccccgacacccgccaacacccgctgacgcgccctgacgggcttgtctgctcccggcatccgcttacagacaagctgtgaccgtctccgggagctgcatgtgtcagaggttttcaccgtcatcaccgaaacgcgcgagacgaaagggcctcgtgatacgcctatttttataggttaatgtcatgataataatggtttcttagacgtcaggtggcacttttcggggaaatgtgcgcggaacccctatttgtttatttttctaaatacattcaaatatgtatccgctcatgagacaataaccctgataaatgcttcaataatattgaaaaaggaagagtcctgaggcggaaagaaccagctgtggaatgtgtgtcagttagggtgtggaaagtccccaggctccccagcaggcagaagtatgcaaagcatgcatctcaattagtcagcaaccaggtgtggaaagtccccaggctccccagcaggcagaagtatgcaaagcatgcatctcaattagtcagcaaccatagtcccgcccctaactccgcccatcccgcccctaactccgcccagttccgcccattctccgccccatggctgactaattttttttatttatgcagaggccgaggccgcctcggcctctgagctattccagaagtagtgaggaggcttttttggaggcctaggcttttgcaaagatcgatcaagagacaggatgaggatcgtttcgcatgattgaacaagatggattgcacgcaggttctccggccgcttgggtggagaggctattcggctatgactgggcacaacagacaatcggctgctctgatgccgccgtgttccggctgtcagcgcaggggcgcccggttctttttgtcaagaccgacctgtccggtgccctgaatgaactgcaagacgaggcagcgcggctatcgtggctggccacgacgggcgttccttgcgcagctgtgctcgacgttgtcactgaagcgggaagggactggctgctattgggcgaagtgccggggcaggatctcctgtcatctcaccttgctcctgccgagaaagtatccatcatggctgatgcaatgcggcggctgcatacgcttgatccggctacctgcccattcgaccaccaagcgaaacatcgcatcgagcgagcacgtactcggatggaagccggtcttgtcgatcaggatgatctggacgaagagcatcaggggctcgcgccagccgaactgttcgccaggctcaaggcgagcatgcccgacggcgaggatctcgtcgtgacccatggcgatgcctgcttgccgaatatcatggtggaaaatggccgcttttctggattcatcgactgtggccggctgggtgtggcggaccgctatcaggacatagcgttggctacccgtgatattgctgaagagcttggcggcgaatgggctgaccgcttcctcgtgctttacggtatcgccgctcccgattcgcagcgcatcgccttctatcgccttcttgacgagttcttctgactgtcagaccaagtttactcatatatactttagattgatttaaaacttcatttttaatttaaaaggatctaggtgaagatcctttttgataatctcatgaccaaaatcccttaacgtgagttttcgttccactgagcgtcagaccccgtagaaaagatcaaaggatcttcttgagatcctttttttctgcgcgtaatctgctgcttgcaaacaaaaaaaccaccgctaccagcggtggtttgtttgccggatcaagagctaccaactctttttccgaaggtaactggcttcagcagagcgcagataccaaatactgttcttctagtgtagccgtagttaggccaccacttcaagaactctgtagcaccgcctacatacctcgctctgctaatcctgttaccagtggctgctgccagtggcgataagtcgtgtcttaccgggttggactcaagacgatagttaccggataaggcgcagcggtcgggctgaacggggggttcgtgcacacagcccagcttggagcgaacgacctacaccgaactgagatacctacagcgtgagctatgagaaagcgccacgcttcccgaagggagaaaggcggacaggtatccggtaagcggcagggtcggaacaggagagcgcacgagggagcttccagggggaaacgcctggtatctttatagtcctgtcgggtttcgccacctctgacttgagcgtcgatttttgtgatgctcgtcaggggggcggagcctatggaaaaacgccagcaacgcggcctttttacggttcctggccttttgctggccttttgctcacatgt

SEQ ID NO: 11 - DNA, 6598 bp, 人工序列（Artificial Sequence）
  pAV-CAG-CYP4V2-P2A-RdCVF-BGH
cctgcaggcagctgcgcgctcgctcgctcactgaggccgcccgggcgtcgggcgacctttggtcgcccggcctcagtgagcgagcgagcgcgcagagagggagtggccaactccatcactaggggttcctgcggccggtcgcgtctagtactagtctagtcgcgtaccattgacgtcaataatgacgtatgttcccatagtaacgccaatagggactttccattgacgtcaatgggtggagtatttacggtaaactgcccacttggcagtacatcaagtgtatcatatgccaagtacgccccctattgacgtcaatgacggtaaatggcccgcctggcattatgcccagtacatgaccttatgggactttcctacttggcagtacatctacgtattagtcatcgctattaccatggtcgaggtgagccccacgttctgcttcactctccccatctcccccccctccccacccccaattttgtatttatttattttttaattattttgtgcagcgatgggggcggggggggggggggggcgcgcgccaggcggggcggggcggggcgaggggcggggcggggcgaggcggagaggtgcggcggcagccaatcagagcggcgcgctccgaaagtttccttttatggcgaggcggcggcggcggcggccctataaaaagcgaagcgcgcggcgggcgggagtcgctgcgacgctgccttcgccccgtgccccgctccgccgccgcctcgcgccgcccgccccggctctgactgaccgcgttactcccacaggtgagcgggcgggacggcccttctcctccgggctgtaattagcgcttggtttaatgacggcttgtttcttttctgtggctgcgtgaaagccttgaggggctccgggagggccctttgtgcggggggagcggctcggggctgtccgcggggggacggctgccttcgggggggacggggcagggcggggttcggcttctggcgtgtgaccggcggctctagagcctctgctaaccatgttcatgccttcttctttttcctacagctcctgggcaacgtgctggttattgtgctgtctcatcattttggcaaagaattggatcggtaccgaggagatctgccaccatggcggggctctggctggggctcgtgtggcagaagctgctgctgtggggcgcggcgagtgccctttccctggccggcgccagtctggtcctgagtctgctgcagagggtggcgagctacgcgcggaaatggcagcagatgcggcccatccccacggtggcccgcgcctacccactggtgggccacgcgctgctgatgaagccggacgggcgagaattttttcagcagatcattgagtacacagaggaataccgccacatgccgctgctgaagctctgggtcgggccagtgcccatggtggccctttataatgcagaaaatgtggaggtaattttaactagttcaaagcaaattgacaaatcctctatgtacaagtttttagaaccatggcttggcctaggacttcttacaagtactggaaacaaatggcgctccaggagaaagatgttaacacccactttccattttaccattctggaagatttcttagatatcatgaatgaacaagcaaatatattggttaagaaacttgaaaaacacattaaccaagaagcatttaactgctttttttacatcactctttgtgccttagatatcatctgtgaaacagctatggggaagaatattggtgctcaaagtaatgatgattccgagtatgtccgtgcagtttatagaatgagtgagatgatatttcgaagaataaagatgccctggctttggcttgatctctggtaccttatgtttaaagaaggatgggaacacaaaaagagccttcagatcctacatacttttaccaacagtgtcatcgcggaacgggccaatgaaatgaacgccaatgaagactgtagaggtgatggcaggggctctgccccctccaaaaataaacgcagggcctttcttgacttgcttttaagtgtgactgatgacgaagggaacaggctaagtcatgaagatattcgagaagaagttgacaccttcatgtttgaggggcacgatacaactgcagctgcaataaactggtccttatacctgttgggttctaacccagaagtccagaaaaaagtggatcatgaattggatgacgtgtttgggaagtctgaccgtcccgctacagtagaagacctgaagaaacttcggtatctggaatgtgttattaaggagacccttcgcctttttccttctgttcctttatttgcccgtagtgttagtgaagattgtgaagtggcaggttacagagttctaaaaggcactgaagccgtcatcattccctatgcattgcacagagatccgagatacttccccaaccccgaggagttccagcctgagcggttcttccccgagaatgcacaagggcgccatccatatgcctacgtgcccttctctgctggccccaggaactgtataggtcaaaagtttgctgtgatggaagaaaagaccattctttcgtgcatcctgaggcacttttggatagaatccaaccagaaaagagaagagcttggtctagaaggacagttgattcttcgtccaagtaatggcatctggatcaagttgaagaggagaaatgcagatgaacgcggaagcggagctactaacttcagcctgctgaagcaggctggagacgtggaggagaaccctggacctatggcctccctgttctctggccgcatcctgatccgcaacaatagcgaccaggacgagctggatacggaggctgaggtcagtcgcaggctggagaaccggctggtgctgctgttctttggtgctggggcttgtccacagtgccaggccttcgtgcccatcctcaaggacttcttcgtgcggctcacagatgagttctatgtactgcgggcggctcagctggccctggtgtacgtgtcccaggactccacggaggagcagcaggacctgttcctcaaggacatgccaaagaaatggcttttcctgccctttgaggatgatctgaggaggtgataaacgcgtggtttatccgatccaccggatctagataagatatccgatccaccggatctagataactgatcataatcagccataccacatttgtagaggttttacttgctttaaaaaacctcccacacctccccctgaacctgaaacataaaatgaatgcaattggcggccgcctcgagctgtgccttctagttgccagccatctgttgtttgcccctcccccgtgccttccttgaccctggaaggtgccactcccactgtcctttcctaataaaatgaggaaattgcatcgcattgtctgagtaggtgtcattctattctggggggtggggtggggcaggacagcaagggggaggattgggaagacaatagcaggcatgctggggatgcggtgggctctatggggtaaccacgtgcggacccaacggccgcaggaacccctagtgatggagttggccactccctctctgcgcgctcgctcgctcactgaggccgggcgaccaaaggtcgcccgacgcccgggctttgcccgggcggcctcagtgagcgagcgagcgcgcagctgcctgcaggggcgcctgatgcggtattttctccttacgcatctgtgcggtatttcacaccgcatacgtcaaagcaaccatagtacgcgccctgtagcggcacattaagcgcggcgggtgtggtggttacgcgcagcgtgaccgctacacttgccagcgccttagcgcccgctcctttcgctttcttcccttcctttctcgccacgttcgccggctttccccgtcaagctctaaatcgggggctccctttagggttccgatttagtgctttacggcacctcgaccccaaaaaacttgatttgggtgatggttcacgtagtgggccatcgccctgatagacggtttttcgccctttgacgttggagtccacgttctttaatagtggactcttgttccaaactggaacaacactcaactctatctcgggctattcttttgatttataagggattttgccgatttcggtctattggttaaaaaatgagctgatttaacaaaaatttaacgcgaattttaacaaaatattaacgtttacaattttatggtgcactctcagtacaatctgctctgatgccgcatagttaagccagccccgacacccgccaacacccgctgacgcgccctgacgggcttgtctgctcccggcatccgcttacagacaagctgtgaccgtctccgggagctgcatgtgtcagaggttttcaccgtcatcaccgaaacgcgcgagacgaaagggcctcgtgatacgcctatttttataggttaatgtcatgataataatggtttcttagacgtcaggtggcacttttcggggaaatgtgcgcggaacccctatttgtttatttttctaaatacattcaaatatgtatccgctcatgagacaataaccctgataaatgcttcaataatattgaaaaaggaagagtcctgaggcggaaagaaccagctgtggaatgtgtgtcagttagggtgtggaaagtccccaggctccccagcaggcagaagtatgcaaagcatgcatctcaattagtcagcaaccaggtgtggaaagtccccaggctccccagcaggcagaagtatgcaaagcatgcatctcaattagtcagcaaccatagtcccgcccctaactccgcccatcccgcccctaactccgcccagttccgcccattctccgccccatggctgactaattttttttatttatgcagaggccgaggccgcctcggcctctgagctattccagaagtagtgaggaggcttttttggaggcctaggcttttgcaaagatcgatcaagagacaggatgaggatcgtttcgcatgattgaacaagatggattgcacgcaggttctccggccgcttgggtggagaggctattcggctatgactgggcacaacagacaatcggctgctctgatgccgccgtgttccggctgtcagcgcaggggcgcccggttctttttgtcaagaccgacctgtccggtgccctgaatgaactgcaagacgaggcagcgcggctatcgtggctggccacgacgggcgttccttgcgcagctgtgctcgacgttgtcactgaagcgggaagggactggctgctattgggcgaagtgccggggcaggatctcctgtcatctcaccttgctcctgccgagaaagtatccatcatggctgatgcaatgcggcggctgcatacgcttgatccggctacctgcccattcgaccaccaagcgaaacatcgcatcgagcgagcacgtactcggatggaagccggtcttgtcgatcaggatgatctggacgaagagcatcaggggctcgcgccagccgaactgttcgccaggctcaaggcgagcatgcccgacggcgaggatctcgtcgtgacccatggcgatgcctgcttgccgaatatcatggtggaaaatggccgcttttctggattcatcgactgtggccggctgggtgtggcggaccgctatcaggacatagcgttggctacccgtgatattgctgaagagcttggcggcgaatgggctgaccgcttcctcgtgctttacggtatcgccgctcccgattcgcagcgcatcgccttctatcgccttcttgacgagttcttctgactgtcagaccaagtttactcatatatactttagattgatttaaaacttcatttttaatttaaaaggatctaggtgaagatcctttttgataatctcatgaccaaaatcccttaacgtgagttttcgttccactgagcgtcagaccccgtagaaaagatcaaaggatcttcttgagatcctttttttctgcgcgtaatctgctgcttgcaaacaaaaaaaccaccgctaccagcggtggtttgtttgccggatcaagagctaccaactctttttccgaaggtaactggcttcagcagagcgcagataccaaatactgttcttctagtgtagccgtagttaggccaccacttcaagaactctgtagcaccgcctacatacctcgctctgctaatcctgttaccagtggctgctgccagtggcgataagtcgtgtcttaccgggttggactcaagacgatagttaccggataaggcgcagcggtcgggctgaacggggggttcgtgcacacagcccagcttggagcgaacgacctacaccgaactgagatacctacagcgtgagctatgagaaagcgccacgcttcccgaagggagaaaggcggacaggtatccggtaagcggcagggtcggaacaggagagcgcacgagggagcttccagggggaaacgcctggtatctttatagtcctgtcgggtttcgccacctctgacttgagcgtcgatttttgtgatgctcgtcaggggggcggagcctatggaaaaacgccagcaacgcggcctttttacggttcctggccttttgctggccttttgctcacatgt

SEQ ID NO: 12 - DNA, 6646 bp, 人工序列（Artificial Sequence）
  pAV-CAG-CYP4V2-P2A-spGL-RdCVF-BGH
cctgcaggcagctgcgcgctcgctcgctcactgaggccgcccgggcgtcgggcgacctttggtcgcccggcctcagtgagcgagcgagcgcgcagagagggagtggccaactccatcactaggggttcctgcggccggtcgcgtctagtactagtctagtcgcgtaccattgacgtcaataatgacgtatgttcccatagtaacgccaatagggactttccattgacgtcaatgggtggagtatttacggtaaactgcccacttggcagtacatcaagtgtatcatatgccaagtacgccccctattgacgtcaatgacggtaaatggcccgcctggcattatgcccagtacatgaccttatgggactttcctacttggcagtacatctacgtattagtcatcgctattaccatggtcgaggtgagccccacgttctgcttcactctccccatctcccccccctccccacccccaattttgtatttatttattttttaattattttgtgcagcgatgggggcggggggggggggggggcgcgcgccaggcggggcggggcggggcgaggggcggggcggggcgaggcggagaggtgcggcggcagccaatcagagcggcgcgctccgaaagtttccttttatggcgaggcggcggcggcggcggccctataaaaagcgaagcgcgcggcgggcgggagtcgctgcgacgctgccttcgccccgtgccccgctccgccgccgcctcgcgccgcccgccccggctctgactgaccgcgttactcccacaggtgagcgggcgggacggcccttctcctccgggctgtaattagcgcttggtttaatgacggcttgtttcttttctgtggctgcgtgaaagccttgaggggctccgggagggccctttgtgcggggggagcggctcggggctgtccgcggggggacggctgccttcgggggggacggggcagggcggggttcggcttctggcgtgtgaccggcggctctagagcctctgctaaccatgttcatgccttcttctttttcctacagctcctgggcaacgtgctggttattgtgctgtctcatcattttggcaaagaattggatcggtaccgaggagatctgccaccatggcggggctctggctggggctcgtgtggcagaagctgctgctgtggggcgcggcgagtgccctttccctggccggcgccagtctggtcctgagtctgctgcagagggtggcgagctacgcgcggaaatggcagcagatgcggcccatccccacggtggcccgcgcctacccactggtgggccacgcgctgctgatgaagccggacgggcgagaattttttcagcagatcattgagtacacagaggaataccgccacatgccgctgctgaagctctgggtcgggccagtgcccatggtggccctttataatgcagaaaatgtggaggtaattttaactagttcaaagcaaattgacaaatcctctatgtacaagtttttagaaccatggcttggcctaggacttcttacaagtactggaaacaaatggcgctccaggagaaagatgttaacacccactttccattttaccattctggaagatttcttagatatcatgaatgaacaagcaaatatattggttaagaaacttgaaaaacacattaaccaagaagcatttaactgctttttttacatcactctttgtgccttagatatcatctgtgaaacagctatggggaagaatattggtgctcaaagtaatgatgattccgagtatgtccgtgcagtttatagaatgagtgagatgatatttcgaagaataaagatgccctggctttggcttgatctctggtaccttatgtttaaagaaggatgggaacacaaaaagagccttcagatcctacatacttttaccaacagtgtcatcgcggaacgggccaatgaaatgaacgccaatgaagactgtagaggtgatggcaggggctctgccccctccaaaaataaacgcagggcctttcttgacttgcttttaagtgtgactgatgacgaagggaacaggctaagtcatgaagatattcgagaagaagttgacaccttcatgtttgaggggcacgatacaactgcagctgcaataaactggtccttatacctgttgggttctaacccagaagtccagaaaaaagtggatcatgaattggatgacgtgtttgggaagtctgaccgtcccgctacagtagaagacctgaagaaacttcggtatctggaatgtgttattaaggagacccttcgcctttttccttctgttcctttatttgcccgtagtgttagtgaagattgtgaagtggcaggttacagagttctaaaaggcactgaagccgtcatcattccctatgcattgcacagagatccgagatacttccccaaccccgaggagttccagcctgagcggttcttccccgagaatgcacaagggcgccatccatatgcctacgtgcccttctctgctggccccaggaactgtataggtcaaaagtttgctgtgatggaagaaaagaccattctttcgtgcatcctgaggcacttttggatagaatccaaccagaaaagagaagagcttggtctagaaggacagttgattcttcgtccaagtaatggcatctggatcaagttgaagaggagaaatgcagatgaacgcggaagcggagctactaacttcagcctgctgaagcaggctggagacgtggaggagaaccctggacctatgggagtcaaagttctgtttgccctgatctgcatcgctgtggccgaggccgcctccctgttctctggccgcatcctgatccgcaacaatagcgaccaggacgagctggatacggaggctgaggtcagtcgcaggctggagaaccggctggtgctgctgttctttggtgctggggcttgtccacagtgccaggccttcgtgcccatcctcaaggacttcttcgtgcggctcacagatgagttctatgtactgcgggcggctcagctggccctggtgtacgtgtcccaggactccacggaggagcagcaggacctgttcctcaaggacatgccaaagaaatggcttttcctgccctttgaggatgatctgaggaggtgataaacgcgtggtttatccgatccaccggatctagataagatatccgatccaccggatctagataactgatcataatcagccataccacatttgtagaggttttacttgctttaaaaaacctcccacacctccccctgaacctgaaacataaaatgaatgcaattggcggccgcctcgagctgtgccttctagttgccagccatctgttgtttgcccctcccccgtgccttccttgaccctggaaggtgccactcccactgtcctttcctaataaaatgaggaaattgcatcgcattgtctgagtaggtgtcattctattctggggggtggggtggggcaggacagcaagggggaggattgggaagacaatagcaggcatgctggggatgcggtgggctctatggggtaaccacgtgcggacccaacggccgcaggaacccctagtgatggagttggccactccctctctgcgcgctcgctcgctcactgaggccgggcgaccaaaggtcgcccgacgcccgggctttgcccgggcggcctcagtgagcgagcgagcgcgcagctgcctgcaggggcgcctgatgcggtattttctccttacgcatctgtgcggtatttcacaccgcatacgtcaaagcaaccatagtacgcgccctgtagcggcacattaagcgcggcgggtgtggtggttacgcgcagcgtgaccgctacacttgccagcgccttagcgcccgctcctttcgctttcttcccttcctttctcgccacgttcgccggctttccccgtcaagctctaaatcgggggctccctttagggttccgatttagtgctttacggcacctcgaccccaaaaaacttgatttgggtgatggttcacgtagtgggccatcgccctgatagacggtttttcgccctttgacgttggagtccacgttctttaatagtggactcttgttccaaactggaacaacactcaactctatctcgggctattcttttgatttataagggattttgccgatttcggtctattggttaaaaaatgagctgatttaacaaaaatttaacgcgaattttaacaaaatattaacgtttacaattttatggtgcactctcagtacaatctgctctgatgccgcatagttaagccagccccgacacccgccaacacccgctgacgcgccctgacgggcttgtctgctcccggcatccgcttacagacaagctgtgaccgtctccgggagctgcatgtgtcagaggttttcaccgtcatcaccgaaacgcgcgagacgaaagggcctcgtgatacgcctatttttataggttaatgtcatgataataatggtttcttagacgtcaggtggcacttttcggggaaatgtgcgcggaacccctatttgtttatttttctaaatacattcaaatatgtatccgctcatgagacaataaccctgataaatgcttcaataatattgaaaaaggaagagtcctgaggcggaaagaaccagctgtggaatgtgtgtcagttagggtgtggaaagtccccaggctccccagcaggcagaagtatgcaaagcatgcatctcaattagtcagcaaccaggtgtggaaagtccccaggctccccagcaggcagaagtatgcaaagcatgcatctcaattagtcagcaaccatagtcccgcccctaactccgcccatcccgcccctaactccgcccagttccgcccattctccgccccatggctgactaattttttttatttatgcagaggccgaggccgcctcggcctctgagctattccagaagtagtgaggaggcttttttggaggcctaggcttttgcaaagatcgatcaagagacaggatgaggatcgtttcgcatgattgaacaagatggattgcacgcaggttctccggccgcttgggtggagaggctattcggctatgactgggcacaacagacaatcggctgctctgatgccgccgtgttccggctgtcagcgcaggggcgcccggttctttttgtcaagaccgacctgtccggtgccctgaatgaactgcaagacgaggcagcgcggctatcgtggctggccacgacgggcgttccttgcgcagctgtgctcgacgttgtcactgaagcgggaagggactggctgctattgggcgaagtgccggggcaggatctcctgtcatctcaccttgctcctgccgagaaagtatccatcatggctgatgcaatgcggcggctgcatacgcttgatccggctacctgcccattcgaccaccaagcgaaacatcgcatcgagcgagcacgtactcggatggaagccggtcttgtcgatcaggatgatctggacgaagagcatcaggggctcgcgccagccgaactgttcgccaggctcaaggcgagcatgcccgacggcgaggatctcgtcgtgacccatggcgatgcctgcttgccgaatatcatggtggaaaatggccgcttttctggattcatcgactgtggccggctgggtgtggcggaccgctatcaggacatagcgttggctacccgtgatattgctgaagagcttggcggcgaatgggctgaccgcttcctcgtgctttacggtatcgccgctcccgattcgcagcgcatcgccttctatcgccttcttgacgagttcttctgactgtcagaccaagtttactcatatatactttagattgatttaaaacttcatttttaatttaaaaggatctaggtgaagatcctttttgataatctcatgaccaaaatcccttaacgtgagttttcgttccactgagcgtcagaccccgtagaaaagatcaaaggatcttcttgagatcctttttttctgcgcgtaatctgctgcttgcaaacaaaaaaaccaccgctaccagcggtggtttgtttgccggatcaagagctaccaactctttttccgaaggtaactggcttcagcagagcgcagataccaaatactgttcttctagtgtagccgtagttaggccaccacttcaagaactctgtagcaccgcctacatacctcgctctgctaatcctgttaccagtggctgctgccagtggcgataagtcgtgtcttaccgggttggactcaagacgatagttaccggataaggcgcagcggtcgggctgaacggggggttcgtgcacacagcccagcttggagcgaacgacctacaccgaactgagatacctacagcgtgagctatgagaaagcgccacgcttcccgaagggagaaaggcggacaggtatccggtaagcggcagggtcggaacaggagagcgcacgagggagcttccagggggaaacgcctggtatctttatagtcctgtcgggtttcgccacctctgacttgagcgtcgatttttgtgatgctcgtcaggggggcggagcctatggaaaaacgccagcaacgcggcctttttacggttcctggccttttgctggccttttgctcacatgt

SEQ ID NO: 13 - DNA, 1863 bp, 人工序列（Artificial Sequence）
  AAV8-CAG-RdCVF
cctgcaggcagctgcgcgctcgctcgctcactgaggccgcccgggcgtcgggcgacctttggtcgcccggcctcagtgagcgagcgagcgcgcagagagggagtggccaactccatcactaggggttcctgcggccggtcgcgtctagtactagtctagtcgcgtaccattgacgtcaataatgacgtatgttcccatagtaacgccaatagggactttccattgacgtcaatgggtggagtatttacggtaaactgcccacttggcagtacatcaagtgtatcatatgccaagtacgccccctattgacgtcaatgacggtaaatggcccgcctggcattatgcccagtacatgaccttatgggactttcctacttggcagtacatctacgtattagtcatcgctattaccatggtcgaggtgagccccacgttctgcttcactctccccatctcccccccctccccacccccaattttgtatttatttattttttaattattttgtgcagcgatgggggcggggggggggggggggcgcgcgccaggcggggcggggcggggcgaggggcggggcggggcgaggcggagaggtgcggcggcagccaatcagagcggcgcgctccgaaagtttccttttatggcgaggcggcggcggcggcggccctataaaaagcgaagcgcgcggcgggcgggagtcgctgcgacgctgccttcgccccgtgccccgctccgccgccgcctcgcgccgcccgccccggctctgactgaccgcgttactcccacaggtgagcgggcgggacggcccttctcctccgggctgtaattagcgcttggtttaatgacggcttgtttcttttctgtggctgcgtgaaagccttgaggggctccgggagggccctttgtgcggggggagcggctcggggctgtccgcggggggacggctgccttcgggggggacggggcagggcggggttcggcttctggcgtgtgaccggcggctctagagcctctgctaaccatgttcatgccttcttctttttcctacagctcctgggcaacgtgctggttattgtgctgtctcatcattttggcaaagaattggatcggtaccgaggagatctgccaccatggcctccctgttctctggccgcatcctgatccgcaacaatagcgaccaggacgagctggatacggaggctgaggtcagtcgcaggctggagaaccggctggtgctgctgttctttggtgctggggcttgtccacagtgccaggccttcgtgcccatcctcaaggacttcttcgtgcggctcacagatgagttctatgtactgcgggcggctcagctggccctggtgtacgtgtcccaggactccacggaggagcagcaggacctgttcctcaaggacatgccaaagaaatggcttttcctgccctttgaggatgatctgaggaggtgataaacgcgtctgtgccttctagttgccagccatctgttgtttgcccctcccccgtgccttccttgaccctggaaggtgccactcccactgtcctttcctaataaaatgaggaaattgcatcgcattgtctgagtaggtgtcattctattctggggggtggggtggggcaggacagcaagggggaggattgggaagacaatagcaggcatgctggggatgcggtgggctctatggggtaaccacgtgcggacccaacggccgcaggaacccctagtgatggagttggccactccctctctgcgcgctcgctcgctcactgaggccgggcgaccaaaggtcgcccgacgcccgggctttgcccgggcggcctcagtgagcgagcgagcgcgcagctgcctgcagg

SEQ ID NO: 14 - DNA, 1911 bp, 人工序列（Artificial Sequence）
  AAV8-CAG-spGL-RdCVF
cctgcaggcagctgcgcgctcgctcgctcactgaggccgcccgggcgtcgggcgacctttggtcgcccggcctcagtgagcgagcgagcgcgcagagagggagtggccaactccatcactaggggttcctgcggccggtcgcgtctagtactagtctagtcgcgtaccattgacgtcaataatgacgtatgttcccatagtaacgccaatagggactttccattgacgtcaatgggtggagtatttacggtaaactgcccacttggcagtacatcaagtgtatcatatgccaagtacgccccctattgacgtcaatgacggtaaatggcccgcctggcattatgcccagtacatgaccttatgggactttcctacttggcagtacatctacgtattagtcatcgctattaccatggtcgaggtgagccccacgttctgcttcactctccccatctcccccccctccccacccccaattttgtatttatttattttttaattattttgtgcagcgatgggggcggggggggggggggggcgcgcgccaggcggggcggggcggggcgaggggcggggcggggcgaggcggagaggtgcggcggcagccaatcagagcggcgcgctccgaaagtttccttttatggcgaggcggcggcggcggcggccctataaaaagcgaagcgcgcggcgggcgggagtcgctgcgacgctgccttcgccccgtgccccgctccgccgccgcctcgcgccgcccgccccggctctgactgaccgcgttactcccacaggtgagcgggcgggacggcccttctcctccgggctgtaattagcgcttggtttaatgacggcttgtttcttttctgtggctgcgtgaaagccttgaggggctccgggagggccctttgtgcggggggagcggctcggggctgtccgcggggggacggctgccttcgggggggacggggcagggcggggttcggcttctggcgtgtgaccggcggctctagagcctctgctaaccatgttcatgccttcttctttttcctacagctcctgggcaacgtgctggttattgtgctgtctcatcattttggcaaagaattggatcggtaccgaggagatctgccaccatgggagtcaaagttctgtttgccctgatctgcatcgctgtggccgaggccgcctccctgttctctggccgcatcctgatccgcaacaatagcgaccaggacgagctggatacggaggctgaggtcagtcgcaggctggagaaccggctggtgctgctgttctttggtgctggggcttgtccacagtgccaggccttcgtgcccatcctcaaggacttcttcgtgcggctcacagatgagttctatgtactgcgggcggctcagctggccctggtgtacgtgtcccaggactccacggaggagcagcaggacctgttcctcaaggacatgccaaagaaatggcttttcctgccctttgaggatgatctgaggaggtgataaacgcgtctgtgccttctagttgccagccatctgttgtttgcccctcccccgtgccttccttgaccctggaaggtgccactcccactgtcctttcctaataaaatgaggaaattgcatcgcattgtctgagtaggtgtcattctattctggggggtggggtggggcaggacagcaagggggaggattgggaagacaatagcaggcatgctggggatgcggtgggctctatggggtaaccacgtgcggacccaacggccgcaggaacccctagtgatggagttggccactccctctctgcgcgctcgctcgctcactgaggccgggcgaccaaaggtcgcccgacgcccgggctttgcccgggcggcctcagtgagcgagcgagcgcgcagctgcctgcagg

SEQ ID NO: 15 - DNA, 51 bp, 人工序列（Artificial Sequence）
  spGL核苷酸
atgggagtcaaagttctgtttgccctgatctgcatcgctgtggccgaggcc

SEQ ID NO: 16 - DNA, 153 bp, 人工序列（Artificial Sequence）
  spGUCY2D核苷酸
atgaccgcctgtgctagaagagccggcggcctccctgatcctggcctgtgcggccctgcttggtgggccccctccctccctagactcccccgggctctgcctagactccccctcctgctcctgctcctgctgctccaaccccccgccctgagc

SEQ ID NO: 17 - DNA, 69 bp, 人工序列（Artificial Sequence）
  spRS1核苷酸
atgagcagaaagatcgagggcttcctgctcctgctcctgttcggctacgaggccaccctgggcctgagc

SEQ ID NO: 18 - DNA, 72 bp, 人工序列（Artificial Sequence）
  spNDP核苷酸
atgagaaagcacgtgctggccgctagcttcagcatgctgagcctgctggtgatcatgggcgacaccgacagc

SEQ ID NO: 19 - DNA, 90 bp, 人工序列（Artificial Sequence）
  spGAS6核苷酸
atggccccctccctgagccccggccccgccgccctcagaagagctcctcagctgctcctgctcctgctggccgccgagtgcgccctggcc

SEQ ID NO: 20 - DNA, 81 bp, 人工序列（Artificial Sequence）
  spCRB1核苷酸
atggccctgaagaacatcaactacctgctgatcttctacctgagcttcagcctgctgatctacatcaagaacagcttctgc

SEQ ID NO: 21 - DNA, 84 bp, 人工序列（Artificial Sequence）
  spCRB2核苷酸
atggccctggctagacctggcacccccgacccccaagccctcgctagcgtcctgctcctgctcctgtgggcccccgccctgagc

SEQ ID NO: 22 - DNA, 327 bp, 人工序列（Artificial Sequence）
  人RdCVF核苷酸
atggcctccctgttctctggccgcatcctgatccgcaacaatagcgaccaggacgagctggatacggaggctgaggtcagtcgcaggctggagaaccggctggtgctgctgttctttggtgctggggcttgtccacagtgccaggccttcgtgcccatcctcaaggacttcttcgtgcggctcacagatgagttctatgtactgcgggcggctcagctggccctggtgtacgtgtcccaggactccacggaggagcagcaggacctgttcctcaaggacatgccaaagaaatggcttttcctgccctttgaggatgatctgaggagg

SEQ ID NO: 23 - DNA, 937 bp, 人工序列（Artificial Sequence）
  CAG核苷酸
ccattgacgtcaataatgacgtatgttcccatagtaacgccaatagggactttccattgacgtcaatgggtggagtatttacggtaaactgcccacttggcagtacatcaagtgtatcatatgccaagtacgccccctattgacgtcaatgacggtaaatggcccgcctggcattatgcccagtacatgaccttatgggactttcctacttggcagtacatctacgtattagtcatcgctattaccatggtcgaggtgagccccacgttctgcttcactctccccatctcccccccctccccacccccaattttgtatttatttattttttaattattttgtgcagcgatgggggcggggggggggggggggcgcgcgccaggcggggcggggcggggcgaggggcggggcggggcgaggcggagaggtgcggcggcagccaatcagagcggcgcgctccgaaagtttccttttatggcgaggcggcggcggcggcggccctataaaaagcgaagcgcgcggcgggcgggagtcgctgcgacgctgccttcgccccgtgccccgctccgccgccgcctcgcgccgcccgccccggctctgactgaccgcgttactcccacaggtgagcgggcgggacggcccttctcctccgggctgtaattagcgcttggtttaatgacggcttgtttcttttctgtggctgcgtgaaagccttgaggggctccgggagggccctttgtgcggggggagcggctcggggctgtccgcggggggacggctgccttcgggggggacggggcagggcggggttcggcttctggcgtgtgaccggcggctctagagcctctgctaaccatgttcatgccttcttctttttcctacagctcctgggcaacgtgctggttattgtgctgtctcatcattttggcaaagaatt

SEQ ID NO: 24 - DNA, 1575 bp, 人工序列（Artificial Sequence）
  CYP4V2核苷酸
atggcggggctctggctggggctcgtgtggcagaagctgctgctgtggggcgcggcgagtgccctttccctggccggcgccagtctggtcctgagtctgctgcagagggtggcgagctacgcgcggaaatggcagcagatgcggcccatccccacggtggcccgcgcctacccactggtgggccacgcgctgctgatgaagccggacgggcgagaattttttcagcagatcattgagtacacagaggaataccgccacatgccgctgctgaagctctgggtcgggccagtgcccatggtggccctttataatgcagaaaatgtggaggtaattttaactagttcaaagcaaattgacaaatcctctatgtacaagtttttagaaccatggcttggcctaggacttcttacaagtactggaaacaaatggcgctccaggagaaagatgttaacacccactttccattttaccattctggaagatttcttagatatcatgaatgaacaagcaaatatattggttaagaaacttgaaaaacacattaaccaagaagcatttaactgctttttttacatcactctttgtgccttagatatcatctgtgaaacagctatggggaagaatattggtgctcaaagtaatgatgattccgagtatgtccgtgcagtttatagaatgagtgagatgatatttcgaagaataaagatgccctggctttggcttgatctctggtaccttatgtttaaagaaggatgggaacacaaaaagagccttcagatcctacatacttttaccaacagtgtcatcgcggaacgggccaatgaaatgaacgccaatgaagactgtagaggtgatggcaggggctctgccccctccaaaaataaacgcagggcctttcttgacttgcttttaagtgtgactgatgacgaagggaacaggctaagtcatgaagatattcgagaagaagttgacaccttcatgtttgaggggcacgatacaactgcagctgcaataaactggtccttatacctgttgggttctaacccagaagtccagaaaaaagtggatcatgaattggatgacgtgtttgggaagtctgaccgtcccgctacagtagaagacctgaagaaacttcggtatctggaatgtgttattaaggagacccttcgcctttttccttctgttcctttatttgcccgtagtgttagtgaagattgtgaagtggcaggttacagagttctaaaaggcactgaagccgtcatcattccctatgcattgcacagagatccgagatacttccccaaccccgaggagttccagcctgagcggttcttccccgagaatgcacaagggcgccatccatatgcctacgtgcccttctctgctggccccaggaactgtataggtcaaaagtttgctgtgatggaagaaaagaccattctttcgtgcatcctgaggcacttttggatagaatccaaccagaaaagagaagagcttggtctagaaggacagttgattcttcgtccaagtaatggcatctggatcaagttgaagaggagaaatgcagatgaacgc

SEQ ID NO: 25 - DNA, 225 bp, 人工序列（Artificial Sequence）
  BGH核苷酸
ctgtgccttctagttgccagccatctgttgtttgcccctcccccgtgccttccttgaccctggaaggtgccactcccactgtcctttcctaataaaatgaggaaattgcatcgcattgtctgagtaggtgtcattctattctggggggtggggtggggcaggacagcaagggggaggattgggaagacaatagcaggcatgctggggatgcggtgggctctatgg

SEQ ID NO: 26 - DNA, 66 bp, 人工序列（Artificial Sequence）
  P2A核苷酸
ggaagcggagctactaacttcagcctgctgaagcaggctggagacgtggaggagaaccctggacct

SEQ ID NO: 27 - protein, 17 aa, 人工序列（Artificial Sequence）
  spGL
MGVKVLFALICIAVAEA

SEQ ID NO: 28 - protein, 51 aa, 人工序列（Artificial Sequence）
  spGUCY2D
MTACARRAGGLPDPGLCGPAWWAPSLPRLPRALPRLPLLLLLLLLQPPALS

SEQ ID NO: 29 - protein, 23 aa, 人工序列（Artificial Sequence）
  spRS1
MSRKIEGFLLLLLFGYEATLGLS

SEQ ID NO: 30 - protein, 24 aa, 人工序列（Artificial Sequence）
  spNDP
MRKHVLAASFSMLSLLVIMGDTDS

SEQ ID NO: 31 - protein, 30 aa, 人工序列（Artificial Sequence）
  spGAS6
MAPSLSPGPAALRRAPQLLLLLLAAECALA

SEQ ID NO: 32 - protein, 27 aa, 人工序列（Artificial Sequence）
  spCRB1
MALKNINYLLIFYLSFSLLIYIKNSFC

SEQ ID NO: 33 - protein, 28 aa, 人工序列（Artificial Sequence）
  spCRB2
MALARPGTPDPQALASVLLLLLWAPALS

SEQ ID NO: 34 - protein, 109 aa, 人类（Homo sapiens）
MASLFSGRILIRNNSDQDELDTEAEVSRRLENRLVLLFFGAGACPQCQAFVPILKDFFVRLTDEFYVLRAAQLALVYVSQDSTEEQQDLFLKDMPKKWLFLPFEDDLRR

SEQ ID NO: 35 - protein, 525 aa, 人类（Homo sapiens）
MAGLWLGLVWQKLLLWGAASALSLAGASLVLSLLQRVASYARKWQQMRPIPTVARAYPLVGHALLMKPDGREFFQQIIEYTEEYRHMPLLKLWVGPVPMVALYNAENVEVILTSSKQIDKSSMYKFLEPWLGLGLLTSTGNKWRSRRKMLTPTFHFTILEDFLDIMNEQANILVKKLEKHINQEAFNCFFYITLCALDIICETAMGKNIGAQSNDDSEYVRAVYRMSEMIFRRIKMPWLWLDLWYLMFKEGWEHKKSLQILHTFTNSVIAERANEMNANEDCRGDGRGSAPSKNKRRAFLDLLLSVTDDEGNRLSHEDIREEVDTFMFEGHDTTAAAINWSLYLLGSNPEVQKKVDHELDDVFGKSDRPATVEDLKKLRYLECVIKETLRLFPSVPLFARSVSEDCEVAGYRVLKGTEAVIIPYALHRDPRYFPNPEEFQPERFFPENAQGRHPYAYVPFSAGPRNCIGQKFAVMEEKTILSCILRHFWIESNQKREELGLEGQLILRPSNGIWIKLKRRNADER

SEQ ID NO: 36 - DNA, 1528 bp, 人工序列（Artificial Sequence）
  CAG-RdCVF-BGH
ccattgacgtcaataatgacgtatgttcccatagtaacgccaatagggactttccattgacgtcaatgggtggagtatttacggtaaactgcccacttggcagtacatcaagtgtatcatatgccaagtacgccccctattgacgtcaatgacggtaaatggcccgcctggcattatgcccagtacatgaccttatgggactttcctacttggcagtacatctacgtattagtcatcgctattaccatggtcgaggtgagccccacgttctgcttcactctccccatctcccccccctccccacccccaattttgtatttatttattttttaattattttgtgcagcgatgggggcggggggggggggggggcgcgcgccaggcggggcggggcggggcgaggggcggggcggggcgaggcggagaggtgcggcggcagccaatcagagcggcgcgctccgaaagtttccttttatggcgaggcggcggcggcggcggccctataaaaagcgaagcgcgcggcgggcgggagtcgctgcgacgctgccttcgccccgtgccccgctccgccgccgcctcgcgccgcccgccccggctctgactgaccgcgttactcccacaggtgagcgggcgggacggcccttctcctccgggctgtaattagcgcttggtttaatgacggcttgtttcttttctgtggctgcgtgaaagccttgaggggctccgggagggccctttgtgcggggggagcggctcggggctgtccgcggggggacggctgccttcgggggggacggggcagggcggggttcggcttctggcgtgtgaccggcggctctagagcctctgctaaccatgttcatgccttcttctttttcctacagctcctgggcaacgtgctggttattgtgctgtctcatcattttggcaaagaattggatcggtaccgaggagatctgccaccatggcctccctgttctctggccgcatcctgatccgcaacaatagcgaccaggacgagctggatacggaggctgaggtcagtcgcaggctggagaaccggctggtgctgctgttctttggtgctggggcttgtccacagtgccaggccttcgtgcccatcctcaaggacttcttcgtgcggctcacagatgagttctatgtactgcgggcggctcagctggccctggtgtacgtgtcccaggactccacggaggagcagcaggacctgttcctcaaggacatgccaaagaaatggcttttcctgccctttgaggatgatctgaggaggtgataaacgcgtctgtgccttctagttgccagccatctgttgtttgcccctcccccgtgccttccttgaccctggaaggtgccactcccactgtcctttcctaataaaatgaggaaattgcatcgcattgtctgagtaggtgtcattctattctggggggtggggtggggcaggacagcaagggggaggattgggaagacaatagcaggcatgctggggatgcggtgggctctatgg

SEQ ID NO: 37 - DNA, 1576 bp, 人工序列（Artificial Sequence）
  CAG-spGL-RdCVF-BGH
ccattgacgtcaataatgacgtatgttcccatagtaacgccaatagggactttccattgacgtcaatgggtggagtatttacggtaaactgcccacttggcagtacatcaagtgtatcatatgccaagtacgccccctattgacgtcaatgacggtaaatggcccgcctggcattatgcccagtacatgaccttatgggactttcctacttggcagtacatctacgtattagtcatcgctattaccatggtcgaggtgagccccacgttctgcttcactctccccatctcccccccctccccacccccaattttgtatttatttattttttaattattttgtgcagcgatgggggcggggggggggggggggcgcgcgccaggcggggcggggcggggcgaggggcggggcggggcgaggcggagaggtgcggcggcagccaatcagagcggcgcgctccgaaagtttccttttatggcgaggcggcggcggcggcggccctataaaaagcgaagcgcgcggcgggcgggagtcgctgcgacgctgccttcgccccgtgccccgctccgccgccgcctcgcgccgcccgccccggctctgactgaccgcgttactcccacaggtgagcgggcgggacggcccttctcctccgggctgtaattagcgcttggtttaatgacggcttgtttcttttctgtggctgcgtgaaagccttgaggggctccgggagggccctttgtgcggggggagcggctcggggctgtccgcggggggacggctgccttcgggggggacggggcagggcggggttcggcttctggcgtgtgaccggcggctctagagcctctgctaaccatgttcatgccttcttctttttcctacagctcctgggcaacgtgctggttattgtgctgtctcatcattttggcaaagaattggatcggtaccgaggagatctgccaccatgggagtcaaagttctgtttgccctgatctgcatcgctgtggccgaggccgcctccctgttctctggccgcatcctgatccgcaacaatagcgaccaggacgagctggatacggaggctgaggtcagtcgcaggctggagaaccggctggtgctgctgttctttggtgctggggcttgtccacagtgccaggccttcgtgcccatcctcaaggacttcttcgtgcggctcacagatgagttctatgtactgcgggcggctcagctggccctggtgtacgtgtcccaggactccacggaggagcagcaggacctgttcctcaaggacatgccaaagaaatggcttttcctgccctttgaggatgatctgaggaggtgataaacgcgtctgtgccttctagttgccagccatctgttgtttgcccctcccccgtgccttccttgaccctggaaggtgccactcccactgtcctttcctaataaaatgaggaaattgcatcgcattgtctgagtaggtgtcattctattctggggggtggggtggggcaggacagcaagggggaggattgggaagacaatagcaggcatgctggggatgcggtgggctctatgg

SEQ ID NO: 38 - DNA, 1678 bp, 人工序列（Artificial Sequence）
  CAG-spGUCY2D-RdCVF-BGH
ccattgacgtcaataatgacgtatgttcccatagtaacgccaatagggactttccattgacgtcaatgggtggagtatttacggtaaactgcccacttggcagtacatcaagtgtatcatatgccaagtacgccccctattgacgtcaatgacggtaaatggcccgcctggcattatgcccagtacatgaccttatgggactttcctacttggcagtacatctacgtattagtcatcgctattaccatggtcgaggtgagccccacgttctgcttcactctccccatctcccccccctccccacccccaattttgtatttatttattttttaattattttgtgcagcgatgggggcggggggggggggggggcgcgcgccaggcggggcggggcggggcgaggggcggggcggggcgaggcggagaggtgcggcggcagccaatcagagcggcgcgctccgaaagtttccttttatggcgaggcggcggcggcggcggccctataaaaagcgaagcgcgcggcgggcgggagtcgctgcgacgctgccttcgccccgtgccccgctccgccgccgcctcgcgccgcccgccccggctctgactgaccgcgttactcccacaggtgagcgggcgggacggcccttctcctccgggctgtaattagcgcttggtttaatgacggcttgtttcttttctgtggctgcgtgaaagccttgaggggctccgggagggccctttgtgcggggggagcggctcggggctgtccgcggggggacggctgccttcgggggggacggggcagggcggggttcggcttctggcgtgtgaccggcggctctagagcctctgctaaccatgttcatgccttcttctttttcctacagctcctgggcaacgtgctggttattgtgctgtctcatcattttggcaaagaattggatcggtaccgaggagatctgccaccatgaccgcctgtgctagaagagccggcggcctccctgatcctggcctgtgcggccctgcttggtgggccccctccctccctagactcccccgggctctgcctagactccccctcctgctcctgctcctgctgctccaaccccccgccctgagcgcctccctgttctctggccgcatcctgatccgcaacaatagcgaccaggacgagctggatacggaggctgaggtcagtcgcaggctggagaaccggctggtgctgctgttctttggtgctggggcttgtccacagtgccaggccttcgtgcccatcctcaaggacttcttcgtgcggctcacagatgagttctatgtactgcgggcggctcagctggccctggtgtacgtgtcccaggactccacggaggagcagcaggacctgttcctcaaggacatgccaaagaaatggcttttcctgccctttgaggatgatctgaggaggtgataaacgcgtctgtgccttctagttgccagccatctgttgtttgcccctcccccgtgccttccttgaccctggaaggtgccactcccactgtcctttcctaataaaatgaggaaattgcatcgcattgtctgagtaggtgtcattctattctggggggtggggtggggcaggacagcaagggggaggattgggaagacaatagcaggcatgctggggatgcggtgggctctatgg

SEQ ID NO: 39 - DNA, 1594 bp, 人工序列（Artificial Sequence）
  CAG-spRS1-RdCVF-BGH
ccattgacgtcaataatgacgtatgttcccatagtaacgccaatagggactttccattgacgtcaatgggtggagtatttacggtaaactgcccacttggcagtacatcaagtgtatcatatgccaagtacgccccctattgacgtcaatgacggtaaatggcccgcctggcattatgcccagtacatgaccttatgggactttcctacttggcagtacatctacgtattagtcatcgctattaccatggtcgaggtgagccccacgttctgcttcactctccccatctcccccccctccccacccccaattttgtatttatttattttttaattattttgtgcagcgatgggggcggggggggggggggggcgcgcgccaggcggggcggggcggggcgaggggcggggcggggcgaggcggagaggtgcggcggcagccaatcagagcggcgcgctccgaaagtttccttttatggcgaggcggcggcggcggcggccctataaaaagcgaagcgcgcggcgggcgggagtcgctgcgacgctgccttcgccccgtgccccgctccgccgccgcctcgcgccgcccgccccggctctgactgaccgcgttactcccacaggtgagcgggcgggacggcccttctcctccgggctgtaattagcgcttggtttaatgacggcttgtttcttttctgtggctgcgtgaaagccttgaggggctccgggagggccctttgtgcggggggagcggctcggggctgtccgcggggggacggctgccttcgggggggacggggcagggcggggttcggcttctggcgtgtgaccggcggctctagagcctctgctaaccatgttcatgccttcttctttttcctacagctcctgggcaacgtgctggttattgtgctgtctcatcattttggcaaagaattggatcggtaccgaggagatctgccaccatgagcagaaagatcgagggcttcctgctcctgctcctgttcggctacgaggccaccctgggcctgagcgcctccctgttctctggccgcatcctgatccgcaacaatagcgaccaggacgagctggatacggaggctgaggtcagtcgcaggctggagaaccggctggtgctgctgttctttggtgctggggcttgtccacagtgccaggccttcgtgcccatcctcaaggacttcttcgtgcggctcacagatgagttctatgtactgcgggcggctcagctggccctggtgtacgtgtcccaggactccacggaggagcagcaggacctgttcctcaaggacatgccaaagaaatggcttttcctgccctttgaggatgatctgaggaggtgataaacgcgtctgtgccttctagttgccagccatctgttgtttgcccctcccccgtgccttccttgaccctggaaggtgccactcccactgtcctttcctaataaaatgaggaaattgcatcgcattgtctgagtaggtgtcattctattctggggggtggggtggggcaggacagcaagggggaggattgggaagacaatagcaggcatgctggggatgcggtgggctctatgg

SEQ ID NO: 40 - DNA, 1597 bp, 人工序列（Artificial Sequence）
  CAG-spNDP-RdCVF-BGH
ccattgacgtcaataatgacgtatgttcccatagtaacgccaatagggactttccattgacgtcaatgggtggagtatttacggtaaactgcccacttggcagtacatcaagtgtatcatatgccaagtacgccccctattgacgtcaatgacggtaaatggcccgcctggcattatgcccagtacatgaccttatgggactttcctacttggcagtacatctacgtattagtcatcgctattaccatggtcgaggtgagccccacgttctgcttcactctccccatctcccccccctccccacccccaattttgtatttatttattttttaattattttgtgcagcgatgggggcggggggggggggggggcgcgcgccaggcggggcggggcggggcgaggggcggggcggggcgaggcggagaggtgcggcggcagccaatcagagcggcgcgctccgaaagtttccttttatggcgaggcggcggcggcggcggccctataaaaagcgaagcgcgcggcgggcgggagtcgctgcgacgctgccttcgccccgtgccccgctccgccgccgcctcgcgccgcccgccccggctctgactgaccgcgttactcccacaggtgagcgggcgggacggcccttctcctccgggctgtaattagcgcttggtttaatgacggcttgtttcttttctgtggctgcgtgaaagccttgaggggctccgggagggccctttgtgcggggggagcggctcggggctgtccgcggggggacggctgccttcgggggggacggggcagggcggggttcggcttctggcgtgtgaccggcggctctagagcctctgctaaccatgttcatgccttcttctttttcctacagctcctgggcaacgtgctggttattgtgctgtctcatcattttggcaaagaattggatcggtaccgaggagatctgccaccatgagaaagcacgtgctggccgctagcttcagcatgctgagcctgctggtgatcatgggcgacaccgacagcgcctccctgttctctggccgcatcctgatccgcaacaatagcgaccaggacgagctggatacggaggctgaggtcagtcgcaggctggagaaccggctggtgctgctgttctttggtgctggggcttgtccacagtgccaggccttcgtgcccatcctcaaggacttcttcgtgcggctcacagatgagttctatgtactgcgggcggctcagctggccctggtgtacgtgtcccaggactccacggaggagcagcaggacctgttcctcaaggacatgccaaagaaatggcttttcctgccctttgaggatgatctgaggaggtgataaacgcgtctgtgccttctagttgccagccatctgttgtttgcccctcccccgtgccttccttgaccctggaaggtgccactcccactgtcctttcctaataaaatgaggaaattgcatcgcattgtctgagtaggtgtcattctattctggggggtggggtggggcaggacagcaagggggaggattgggaagacaatagcaggcatgctggggatgcggtgggctctatgg

SEQ ID NO: 41 - DNA, 1615 bp, 人工序列（Artificial Sequence）
  CAG-spGAS6-RdCVF-BGH
ccattgacgtcaataatgacgtatgttcccatagtaacgccaatagggactttccattgacgtcaatgggtggagtatttacggtaaactgcccacttggcagtacatcaagtgtatcatatgccaagtacgccccctattgacgtcaatgacggtaaatggcccgcctggcattatgcccagtacatgaccttatgggactttcctacttggcagtacatctacgtattagtcatcgctattaccatggtcgaggtgagccccacgttctgcttcactctccccatctcccccccctccccacccccaattttgtatttatttattttttaattattttgtgcagcgatgggggcggggggggggggggggcgcgcgccaggcggggcggggcggggcgaggggcggggcggggcgaggcggagaggtgcggcggcagccaatcagagcggcgcgctccgaaagtttccttttatggcgaggcggcggcggcggcggccctataaaaagcgaagcgcgcggcgggcgggagtcgctgcgacgctgccttcgccccgtgccccgctccgccgccgcctcgcgccgcccgccccggctctgactgaccgcgttactcccacaggtgagcgggcgggacggcccttctcctccgggctgtaattagcgcttggtttaatgacggcttgtttcttttctgtggctgcgtgaaagccttgaggggctccgggagggccctttgtgcggggggagcggctcggggctgtccgcggggggacggctgccttcgggggggacggggcagggcggggttcggcttctggcgtgtgaccggcggctctagagcctctgctaaccatgttcatgccttcttctttttcctacagctcctgggcaacgtgctggttattgtgctgtctcatcattttggcaaagaattggatcggtaccgaggagatctgccaccatggccccctccctgagccccggccccgccgccctcagaagagctcctcagctgctcctgctcctgctggccgccgagtgcgccctggccgcctccctgttctctggccgcatcctgatccgcaacaatagcgaccaggacgagctggatacggaggctgaggtcagtcgcaggctggagaaccggctggtgctgctgttctttggtgctggggcttgtccacagtgccaggccttcgtgcccatcctcaaggacttcttcgtgcggctcacagatgagttctatgtactgcgggcggctcagctggccctggtgtacgtgtcccaggactccacggaggagcagcaggacctgttcctcaaggacatgccaaagaaatggcttttcctgccctttgaggatgatctgaggaggtgataaacgcgtctgtgccttctagttgccagccatctgttgtttgcccctcccccgtgccttccttgaccctggaaggtgccactcccactgtcctttcctaataaaatgaggaaattgcatcgcattgtctgagtaggtgtcattctattctggggggtggggtggggcaggacagcaagggggaggattgggaagacaatagcaggcatgctggggatgcggtgggctctatgg

SEQ ID NO: 42 - DNA, 1606 bp, 人工序列（Artificial Sequence）
  CAG-spCRB1-RdCVF-BGH
ccattgacgtcaataatgacgtatgttcccatagtaacgccaatagggactttccattgacgtcaatgggtggagtatttacggtaaactgcccacttggcagtacatcaagtgtatcatatgccaagtacgccccctattgacgtcaatgacggtaaatggcccgcctggcattatgcccagtacatgaccttatgggactttcctacttggcagtacatctacgtattagtcatcgctattaccatggtcgaggtgagccccacgttctgcttcactctccccatctcccccccctccccacccccaattttgtatttatttattttttaattattttgtgcagcgatgggggcggggggggggggggggcgcgcgccaggcggggcggggcggggcgaggggcggggcggggcgaggcggagaggtgcggcggcagccaatcagagcggcgcgctccgaaagtttccttttatggcgaggcggcggcggcggcggccctataaaaagcgaagcgcgcggcgggcgggagtcgctgcgacgctgccttcgccccgtgccccgctccgccgccgcctcgcgccgcccgccccggctctgactgaccgcgttactcccacaggtgagcgggcgggacggcccttctcctccgggctgtaattagcgcttggtttaatgacggcttgtttcttttctgtggctgcgtgaaagccttgaggggctccgggagggccctttgtgcggggggagcggctcggggctgtccgcggggggacggctgccttcgggggggacggggcagggcggggttcggcttctggcgtgtgaccggcggctctagagcctctgctaaccatgttcatgccttcttctttttcctacagctcctgggcaacgtgctggttattgtgctgtctcatcattttggcaaagaattggatcggtaccgaggagatctgccaccatggccctgaagaacatcaactacctgctgatcttctacctgagcttcagcctgctgatctacatcaagaacagcttctgcgcctccctgttctctggccgcatcctgatccgcaacaatagcgaccaggacgagctggatacggaggctgaggtcagtcgcaggctggagaaccggctggtgctgctgttctttggtgctggggcttgtccacagtgccaggccttcgtgcccatcctcaaggacttcttcgtgcggctcacagatgagttctatgtactgcgggcggctcagctggccctggtgtacgtgtcccaggactccacggaggagcagcaggacctgttcctcaaggacatgccaaagaaatggcttttcctgccctttgaggatgatctgaggaggtgataaacgcgtctgtgccttctagttgccagccatctgttgtttgcccctcccccgtgccttccttgaccctggaaggtgccactcccactgtcctttcctaataaaatgaggaaattgcatcgcattgtctgagtaggtgtcattctattctggggggtggggtggggcaggacagcaagggggaggattgggaagacaatagcaggcatgctggggatgcggtgggctctatgg

SEQ ID NO: 43 - DNA, 1609 bp, 人工序列（Artificial Sequence）
  CAG-spCRB2-RdCVF-BGH
ccattgacgtcaataatgacgtatgttcccatagtaacgccaatagggactttccattgacgtcaatgggtggagtatttacggtaaactgcccacttggcagtacatcaagtgtatcatatgccaagtacgccccctattgacgtcaatgacggtaaatggcccgcctggcattatgcccagtacatgaccttatgggactttcctacttggcagtacatctacgtattagtcatcgctattaccatggtcgaggtgagccccacgttctgcttcactctccccatctcccccccctccccacccccaattttgtatttatttattttttaattattttgtgcagcgatgggggcggggggggggggggggcgcgcgccaggcggggcggggcggggcgaggggcggggcggggcgaggcggagaggtgcggcggcagccaatcagagcggcgcgctccgaaagtttccttttatggcgaggcggcggcggcggcggccctataaaaagcgaagcgcgcggcgggcgggagtcgctgcgacgctgccttcgccccgtgccccgctccgccgccgcctcgcgccgcccgccccggctctgactgaccgcgttactcccacaggtgagcgggcgggacggcccttctcctccgggctgtaattagcgcttggtttaatgacggcttgtttcttttctgtggctgcgtgaaagccttgaggggctccgggagggccctttgtgcggggggagcggctcggggctgtccgcggggggacggctgccttcgggggggacggggcagggcggggttcggcttctggcgtgtgaccggcggctctagagcctctgctaaccatgttcatgccttcttctttttcctacagctcctgggcaacgtgctggttattgtgctgtctcatcattttggcaaagaattggatcggtaccgaggagatctgccaccatggccctggctagacctggcacccccgacccccaagccctcgctagcgtcctgctcctgctcctgtgggcccccgccctgagcgcctccctgttctctggccgcatcctgatccgcaacaatagcgaccaggacgagctggatacggaggctgaggtcagtcgcaggctggagaaccggctggtgctgctgttctttggtgctggggcttgtccacagtgccaggccttcgtgcccatcctcaaggacttcttcgtgcggctcacagatgagttctatgtactgcgggcggctcagctggccctggtgtacgtgtcccaggactccacggaggagcagcaggacctgttcctcaaggacatgccaaagaaatggcttttcctgccctttgaggatgatctgaggaggtgataaacgcgtctgtgccttctagttgccagccatctgttgtttgcccctcccccgtgccttccttgaccctggaaggtgccactcccactgtcctttcctaataaaatgaggaaattgcatcgcattgtctgagtaggtgtcattctattctggggggtggggtggggcaggacagcaagggggaggattgggaagacaatagcaggcatgctggggatgcggtgggctctatgg

SEQ ID NO: 44 - DNA, 4469 bp, 人工序列（Artificial Sequence）
  CAG-CYP4V2-BGH-CAG-RdCVF-BGH
ccattgacgtcaataatgacgtatgttcccatagtaacgccaatagggactttccattgacgtcaatgggtggagtatttacggtaaactgcccacttggcagtacatcaagtgtatcatatgccaagtacgccccctattgacgtcaatgacggtaaatggcccgcctggcattatgcccagtacatgaccttatgggactttcctacttggcagtacatctacgtattagtcatcgctattaccatggtcgaggtgagccccacgttctgcttcactctccccatctcccccccctccccacccccaattttgtatttatttattttttaattattttgtgcagcgatgggggcggggggggggggggggcgcgcgccaggcggggcggggcggggcgaggggcggggcggggcgaggcggagaggtgcggcggcagccaatcagagcggcgcgctccgaaagtttccttttatggcgaggcggcggcggcggcggccctataaaaagcgaagcgcgcggcgggcgggagtcgctgcgacgctgccttcgccccgtgccccgctccgccgccgcctcgcgccgcccgccccggctctgactgaccgcgttactcccacaggtgagcgggcgggacggcccttctcctccgggctgtaattagcgcttggtttaatgacggcttgtttcttttctgtggctgcgtgaaagccttgaggggctccgggagggccctttgtgcggggggagcggctcggggctgtccgcggggggacggctgccttcgggggggacggggcagggcggggttcggcttctggcgtgtgaccggcggctctagagcctctgctaaccatgttcatgccttcttctttttcctacagctcctgggcaacgtgctggttattgtgctgtctcatcattttggcaaagaattggatcggtaccgaggagatctgccaccatggcggggctctggctggggctcgtgtggcagaagctgctgctgtggggcgcggcgagtgccctttccctggccggcgccagtctggtcctgagtctgctgcagagggtggcgagctacgcgcggaaatggcagcagatgcggcccatccccacggtggcccgcgcctacccactggtgggccacgcgctgctgatgaagccggacgggcgagaattttttcagcagatcattgagtacacagaggaataccgccacatgccgctgctgaagctctgggtcgggccagtgcccatggtggccctttataatgcagaaaatgtggaggtaattttaactagttcaaagcaaattgacaaatcctctatgtacaagtttttagaaccatggcttggcctaggacttcttacaagtactggaaacaaatggcgctccaggagaaagatgttaacacccactttccattttaccattctggaagatttcttagatatcatgaatgaacaagcaaatatattggttaagaaacttgaaaaacacattaaccaagaagcatttaactgctttttttacatcactctttgtgccttagatatcatctgtgaaacagctatggggaagaatattggtgctcaaagtaatgatgattccgagtatgtccgtgcagtttatagaatgagtgagatgatatttcgaagaataaagatgccctggctttggcttgatctctggtaccttatgtttaaagaaggatgggaacacaaaaagagccttcagatcctacatacttttaccaacagtgtcatcgcggaacgggccaatgaaatgaacgccaatgaagactgtagaggtgatggcaggggctctgccccctccaaaaataaacgcagggcctttcttgacttgcttttaagtgtgactgatgacgaagggaacaggctaagtcatgaagatattcgagaagaagttgacaccttcatgtttgaggggcacgatacaactgcagctgcaataaactggtccttatacctgttgggttctaacccagaagtccagaaaaaagtggatcatgaattggatgacgtgtttgggaagtctgaccgtcccgctacagtagaagacctgaagaaacttcggtatctggaatgtgttattaaggagacccttcgcctttttccttctgttcctttatttgcccgtagtgttagtgaagattgtgaagtggcaggttacagagttctaaaaggcactgaagccgtcatcattccctatgcattgcacagagatccgagatacttccccaaccccgaggagttccagcctgagcggttcttccccgagaatgcacaagggcgccatccatatgcctacgtgcccttctctgctggccccaggaactgtataggtcaaaagtttgctgtgatggaagaaaagaccattctttcgtgcatcctgaggcacttttggatagaatccaaccagaaaagagaagagcttggtctagaaggacagttgattcttcgtccaagtaatggcatctggatcaagttgaagaggagaaatgcagatgaacgctaaacgcgtggtttatccgatccaccggatctagataagatatccgatccaccggatctagataactgatcataatcagccataccacatttgtagaggttttacttgctttaaaaaacctcccacacctccccctgaacctgaaacataaaatgaatgcaattggcggccgcctcgagctgtgccttctagttgccagccatctgttgtttgcccctcccccgtgccttccttgaccctggaaggtgccactcccactgtcctttcctaataaaatgaggaaattgcatcgcattgtctgagtaggtgtcattctattctggggggtggggtggggcaggacagcaagggggaggattgggaagacaatagcaggcatgctggggatgcggtgggctctatggggtaaccccattgacgtcaataatgacgtatgttcccatagtaacgccaatagggactttccattgacgtcaatgggtggagtatttacggtaaactgcccacttggcagtacatcaagtgtatcatatgccaagtacgccccctattgacgtcaatgacggtaaatggcccgcctggcattatgcccagtacatgaccttatgggactttcctacttggcagtacatctacgtattagtcatcgctattaccatggtcgaggtgagccccacgttctgcttcactctccccatctcccccccctccccacccccaattttgtatttatttattttttaattattttgtgcagcgatgggggcggggggggggggggggcgcgcgccaggcggggcggggcggggcgaggggcggggcggggcgaggcggagaggtgcggcggcagccaatcagagcggcgcgctccgaaagtttccttttatggcgaggcggcggcggcggcggccctataaaaagcgaagcgcgcggcgggcgggagtcgctgcgacgctgccttcgccccgtgccccgctccgccgccgcctcgcgccgcccgccccggctctgactgaccgcgttactcccacaggtgagcgggcgggacggcccttctcctccgggctgtaattagcgcttggtttaatgacggcttgtttcttttctgtggctgcgtgaaagccttgaggggctccgggagggccctttgtgcggggggagcggctcggggctgtccgcggggggacggctgccttcgggggggacggggcagggcggggttcggcttctggcgtgtgaccggcggctctagagcctctgctaaccatgttcatgccttcttctttttcctacagctcctgggcaacgtgctggttattgtgctgtctcatcattttggcaaagaattggatcggtaccgaggagatctgccaccatggcctccctgttctctggccgcatcctgatccgcaacaatagcgaccaggacgagctggatacggaggctgaggtcagtcgcaggctggagaaccggctggtgctgctgttctttggtgctggggcttgtccacagtgccaggccttcgtgcccatcctcaaggacttcttcgtgcggctcacagatgagttctatgtactgcgggcggctcagctggccctggtgtacgtgtcccaggactccacggaggagcagcaggacctgttcctcaaggacatgccaaagaaatggcttttcctgccctttgaggatgatctgaggaggtgactgtgccttctagttgccagccatctgttgtttgcccctcccccgtgccttccttgaccctggaaggtgccactcccactgtcctttcctaataaaatgaggaaattgcatcgcattgtctgagtaggtgtcattctattctggggggtggggtggggcaggacagcaagggggaggattgggaagacaatagcaggcatgctggggatgcggtgggctctatgg

SEQ ID NO: 45 - DNA, 4517 bp, 人工序列（Artificial Sequence）
  CAG-CYP4V2-BGH-CAG-spGL-RdCVF-BGH
ccattgacgtcaataatgacgtatgttcccatagtaacgccaatagggactttccattgacgtcaatgggtggagtatttacggtaaactgcccacttggcagtacatcaagtgtatcatatgccaagtacgccccctattgacgtcaatgacggtaaatggcccgcctggcattatgcccagtacatgaccttatgggactttcctacttggcagtacatctacgtattagtcatcgctattaccatggtcgaggtgagccccacgttctgcttcactctccccatctcccccccctccccacccccaattttgtatttatttattttttaattattttgtgcagcgatgggggcggggggggggggggggcgcgcgccaggcggggcggggcggggcgaggggcggggcggggcgaggcggagaggtgcggcggcagccaatcagagcggcgcgctccgaaagtttccttttatggcgaggcggcggcggcggcggccctataaaaagcgaagcgcgcggcgggcgggagtcgctgcgacgctgccttcgccccgtgccccgctccgccgccgcctcgcgccgcccgccccggctctgactgaccgcgttactcccacaggtgagcgggcgggacggcccttctcctccgggctgtaattagcgcttggtttaatgacggcttgtttcttttctgtggctgcgtgaaagccttgaggggctccgggagggccctttgtgcggggggagcggctcggggctgtccgcggggggacggctgccttcgggggggacggggcagggcggggttcggcttctggcgtgtgaccggcggctctagagcctctgctaaccatgttcatgccttcttctttttcctacagctcctgggcaacgtgctggttattgtgctgtctcatcattttggcaaagaattggatcggtaccgaggagatctgccaccatggcggggctctggctggggctcgtgtggcagaagctgctgctgtggggcgcggcgagtgccctttccctggccggcgccagtctggtcctgagtctgctgcagagggtggcgagctacgcgcggaaatggcagcagatgcggcccatccccacggtggcccgcgcctacccactggtgggccacgcgctgctgatgaagccggacgggcgagaattttttcagcagatcattgagtacacagaggaataccgccacatgccgctgctgaagctctgggtcgggccagtgcccatggtggccctttataatgcagaaaatgtggaggtaattttaactagttcaaagcaaattgacaaatcctctatgtacaagtttttagaaccatggcttggcctaggacttcttacaagtactggaaacaaatggcgctccaggagaaagatgttaacacccactttccattttaccattctggaagatttcttagatatcatgaatgaacaagcaaatatattggttaagaaacttgaaaaacacattaaccaagaagcatttaactgctttttttacatcactctttgtgccttagatatcatctgtgaaacagctatggggaagaatattggtgctcaaagtaatgatgattccgagtatgtccgtgcagtttatagaatgagtgagatgatatttcgaagaataaagatgccctggctttggcttgatctctggtaccttatgtttaaagaaggatgggaacacaaaaagagccttcagatcctacatacttttaccaacagtgtcatcgcggaacgggccaatgaaatgaacgccaatgaagactgtagaggtgatggcaggggctctgccccctccaaaaataaacgcagggcctttcttgacttgcttttaagtgtgactgatgacgaagggaacaggctaagtcatgaagatattcgagaagaagttgacaccttcatgtttgaggggcacgatacaactgcagctgcaataaactggtccttatacctgttgggttctaacccagaagtccagaaaaaagtggatcatgaattggatgacgtgtttgggaagtctgaccgtcccgctacagtagaagacctgaagaaacttcggtatctggaatgtgttattaaggagacccttcgcctttttccttctgttcctttatttgcccgtagtgttagtgaagattgtgaagtggcaggttacagagttctaaaaggcactgaagccgtcatcattccctatgcattgcacagagatccgagatacttccccaaccccgaggagttccagcctgagcggttcttccccgagaatgcacaagggcgccatccatatgcctacgtgcccttctctgctggccccaggaactgtataggtcaaaagtttgctgtgatggaagaaaagaccattctttcgtgcatcctgaggcacttttggatagaatccaaccagaaaagagaagagcttggtctagaaggacagttgattcttcgtccaagtaatggcatctggatcaagttgaagaggagaaatgcagatgaacgctaaacgcgtggtttatccgatccaccggatctagataagatatccgatccaccggatctagataactgatcataatcagccataccacatttgtagaggttttacttgctttaaaaaacctcccacacctccccctgaacctgaaacataaaatgaatgcaattggcggccgcctcgagctgtgccttctagttgccagccatctgttgtttgcccctcccccgtgccttccttgaccctggaaggtgccactcccactgtcctttcctaataaaatgaggaaattgcatcgcattgtctgagtaggtgtcattctattctggggggtggggtggggcaggacagcaagggggaggattgggaagacaatagcaggcatgctggggatgcggtgggctctatggggtaaccccattgacgtcaataatgacgtatgttcccatagtaacgccaatagggactttccattgacgtcaatgggtggagtatttacggtaaactgcccacttggcagtacatcaagtgtatcatatgccaagtacgccccctattgacgtcaatgacggtaaatggcccgcctggcattatgcccagtacatgaccttatgggactttcctacttggcagtacatctacgtattagtcatcgctattaccatggtcgaggtgagccccacgttctgcttcactctccccatctcccccccctccccacccccaattttgtatttatttattttttaattattttgtgcagcgatgggggcggggggggggggggggcgcgcgccaggcggggcggggcggggcgaggggcggggcggggcgaggcggagaggtgcggcggcagccaatcagagcggcgcgctccgaaagtttccttttatggcgaggcggcggcggcggcggccctataaaaagcgaagcgcgcggcgggcgggagtcgctgcgacgctgccttcgccccgtgccccgctccgccgccgcctcgcgccgcccgccccggctctgactgaccgcgttactcccacaggtgagcgggcgggacggcccttctcctccgggctgtaattagcgcttggtttaatgacggcttgtttcttttctgtggctgcgtgaaagccttgaggggctccgggagggccctttgtgcggggggagcggctcggggctgtccgcggggggacggctgccttcgggggggacggggcagggcggggttcggcttctggcgtgtgaccggcggctctagagcctctgctaaccatgttcatgccttcttctttttcctacagctcctgggcaacgtgctggttattgtgctgtctcatcattttggcaaagaattggatcggtaccgaggagatctgccaccatgggagtcaaagttctgtttgccctgatctgcatcgctgtggccgaggccgcctccctgttctctggccgcatcctgatccgcaacaatagcgaccaggacgagctggatacggaggctgaggtcagtcgcaggctggagaaccggctggtgctgctgttctttggtgctggggcttgtccacagtgccaggccttcgtgcccatcctcaaggacttcttcgtgcggctcacagatgagttctatgtactgcgggcggctcagctggccctggtgtacgtgtcccaggactccacggaggagcagcaggacctgttcctcaaggacatgccaaagaaatggcttttcctgccctttgaggatgatctgaggaggtgactgtgccttctagttgccagccatctgttgtttgcccctcccccgtgccttccttgaccctggaaggtgccactcccactgtcctttcctaataaaatgaggaaattgcatcgcattgtctgagtaggtgtcattctattctggggggtggggtggggcaggacagcaagggggaggattgggaagacaatagcaggcatgctggggatgcggtgggctctatgg

SEQ ID NO: 46 - DNA, 3339 bp, 人工序列（Artificial Sequence）
  CAG-CYP4V2-P2A-RdCVF-BGH
ccattgacgtcaataatgacgtatgttcccatagtaacgccaatagggactttccattgacgtcaatgggtggagtatttacggtaaactgcccacttggcagtacatcaagtgtatcatatgccaagtacgccccctattgacgtcaatgacggtaaatggcccgcctggcattatgcccagtacatgaccttatgggactttcctacttggcagtacatctacgtattagtcatcgctattaccatggtcgaggtgagccccacgttctgcttcactctccccatctcccccccctccccacccccaattttgtatttatttattttttaattattttgtgcagcgatgggggcggggggggggggggggcgcgcgccaggcggggcggggcggggcgaggggcggggcggggcgaggcggagaggtgcggcggcagccaatcagagcggcgcgctccgaaagtttccttttatggcgaggcggcggcggcggcggccctataaaaagcgaagcgcgcggcgggcgggagtcgctgcgacgctgccttcgccccgtgccccgctccgccgccgcctcgcgccgcccgccccggctctgactgaccgcgttactcccacaggtgagcgggcgggacggcccttctcctccgggctgtaattagcgcttggtttaatgacggcttgtttcttttctgtggctgcgtgaaagccttgaggggctccgggagggccctttgtgcggggggagcggctcggggctgtccgcggggggacggctgccttcgggggggacggggcagggcggggttcggcttctggcgtgtgaccggcggctctagagcctctgctaaccatgttcatgccttcttctttttcctacagctcctgggcaacgtgctggttattgtgctgtctcatcattttggcaaagaattggatcggtaccgaggagatctgccaccatggcggggctctggctggggctcgtgtggcagaagctgctgctgtggggcgcggcgagtgccctttccctggccggcgccagtctggtcctgagtctgctgcagagggtggcgagctacgcgcggaaatggcagcagatgcggcccatccccacggtggcccgcgcctacccactggtgggccacgcgctgctgatgaagccggacgggcgagaattttttcagcagatcattgagtacacagaggaataccgccacatgccgctgctgaagctctgggtcgggccagtgcccatggtggccctttataatgcagaaaatgtggaggtaattttaactagttcaaagcaaattgacaaatcctctatgtacaagtttttagaaccatggcttggcctaggacttcttacaagtactggaaacaaatggcgctccaggagaaagatgttaacacccactttccattttaccattctggaagatttcttagatatcatgaatgaacaagcaaatatattggttaagaaacttgaaaaacacattaaccaagaagcatttaactgctttttttacatcactctttgtgccttagatatcatctgtgaaacagctatggggaagaatattggtgctcaaagtaatgatgattccgagtatgtccgtgcagtttatagaatgagtgagatgatatttcgaagaataaagatgccctggctttggcttgatctctggtaccttatgtttaaagaaggatgggaacacaaaaagagccttcagatcctacatacttttaccaacagtgtcatcgcggaacgggccaatgaaatgaacgccaatgaagactgtagaggtgatggcaggggctctgccccctccaaaaataaacgcagggcctttcttgacttgcttttaagtgtgactgatgacgaagggaacaggctaagtcatgaagatattcgagaagaagttgacaccttcatgtttgaggggcacgatacaactgcagctgcaataaactggtccttatacctgttgggttctaacccagaagtccagaaaaaagtggatcatgaattggatgacgtgtttgggaagtctgaccgtcccgctacagtagaagacctgaagaaacttcggtatctggaatgtgttattaaggagacccttcgcctttttccttctgttcctttatttgcccgtagtgttagtgaagattgtgaagtggcaggttacagagttctaaaaggcactgaagccgtcatcattccctatgcattgcacagagatccgagatacttccccaaccccgaggagttccagcctgagcggttcttccccgagaatgcacaagggcgccatccatatgcctacgtgcccttctctgctggccccaggaactgtataggtcaaaagtttgctgtgatggaagaaaagaccattctttcgtgcatcctgaggcacttttggatagaatccaaccagaaaagagaagagcttggtctagaaggacagttgattcttcgtccaagtaatggcatctggatcaagttgaagaggagaaatgcagatgaacgcggaagcggagctactaacttcagcctgctgaagcaggctggagacgtggaggagaaccctggacctatggcctccctgttctctggccgcatcctgatccgcaacaatagcgaccaggacgagctggatacggaggctgaggtcagtcgcaggctggagaaccggctggtgctgctgttctttggtgctggggcttgtccacagtgccaggccttcgtgcccatcctcaaggacttcttcgtgcggctcacagatgagttctatgtactgcgggcggctcagctggccctggtgtacgtgtcccaggactccacggaggagcagcaggacctgttcctcaaggacatgccaaagaaatggcttttcctgccctttgaggatgatctgaggaggtgataaacgcgtggtttatccgatccaccggatctagataagatatccgatccaccggatctagataactgatcataatcagccataccacatttgtagaggttttacttgctttaaaaaacctcccacacctccccctgaacctgaaacataaaatgaatgcaattggcggccgcctcgagctgtgccttctagttgccagccatctgttgtttgcccctcccccgtgccttccttgaccctggaaggtgccactcccactgtcctttcctaataaaatgaggaaattgcatcgcattgtctgagtaggtgtcattctattctggggggtggggtggggcaggacagcaagggggaggattgggaagacaatagcaggcatgctggggatgcggtgggctctatgg

SEQ ID NO: 47 - DNA, 3387 bp, 人工序列（Artificial Sequence）
  CAG-CYP4V2-P2A-spGL-RdCVF-BGH
ccattgacgtcaataatgacgtatgttcccatagtaacgccaatagggactttccattgacgtcaatgggtggagtatttacggtaaactgcccacttggcagtacatcaagtgtatcatatgccaagtacgccccctattgacgtcaatgacggtaaatggcccgcctggcattatgcccagtacatgaccttatgggactttcctacttggcagtacatctacgtattagtcatcgctattaccatggtcgaggtgagccccacgttctgcttcactctccccatctcccccccctccccacccccaattttgtatttatttattttttaattattttgtgcagcgatgggggcggggggggggggggggcgcgcgccaggcggggcggggcggggcgaggggcggggcggggcgaggcggagaggtgcggcggcagccaatcagagcggcgcgctccgaaagtttccttttatggcgaggcggcggcggcggcggccctataaaaagcgaagcgcgcggcgggcgggagtcgctgcgacgctgccttcgccccgtgccccgctccgccgccgcctcgcgccgcccgccccggctctgactgaccgcgttactcccacaggtgagcgggcgggacggcccttctcctccgggctgtaattagcgcttggtttaatgacggcttgtttcttttctgtggctgcgtgaaagccttgaggggctccgggagggccctttgtgcggggggagcggctcggggctgtccgcggggggacggctgccttcgggggggacggggcagggcggggttcggcttctggcgtgtgaccggcggctctagagcctctgctaaccatgttcatgccttcttctttttcctacagctcctgggcaacgtgctggttattgtgctgtctcatcattttggcaaagaattggatcggtaccgaggagatctgccaccatggcggggctctggctggggctcgtgtggcagaagctgctgctgtggggcgcggcgagtgccctttccctggccggcgccagtctggtcctgagtctgctgcagagggtggcgagctacgcgcggaaatggcagcagatgcggcccatccccacggtggcccgcgcctacccactggtgggccacgcgctgctgatgaagccggacgggcgagaattttttcagcagatcattgagtacacagaggaataccgccacatgccgctgctgaagctctgggtcgggccagtgcccatggtggccctttataatgcagaaaatgtggaggtaattttaactagttcaaagcaaattgacaaatcctctatgtacaagtttttagaaccatggcttggcctaggacttcttacaagtactggaaacaaatggcgctccaggagaaagatgttaacacccactttccattttaccattctggaagatttcttagatatcatgaatgaacaagcaaatatattggttaagaaacttgaaaaacacattaaccaagaagcatttaactgctttttttacatcactctttgtgccttagatatcatctgtgaaacagctatggggaagaatattggtgctcaaagtaatgatgattccgagtatgtccgtgcagtttatagaatgagtgagatgatatttcgaagaataaagatgccctggctttggcttgatctctggtaccttatgtttaaagaaggatgggaacacaaaaagagccttcagatcctacatacttttaccaacagtgtcatcgcggaacgggccaatgaaatgaacgccaatgaagactgtagaggtgatggcaggggctctgccccctccaaaaataaacgcagggcctttcttgacttgcttttaagtgtgactgatgacgaagggaacaggctaagtcatgaagatattcgagaagaagttgacaccttcatgtttgaggggcacgatacaactgcagctgcaataaactggtccttatacctgttgggttctaacccagaagtccagaaaaaagtggatcatgaattggatgacgtgtttgggaagtctgaccgtcccgctacagtagaagacctgaagaaacttcggtatctggaatgtgttattaaggagacccttcgcctttttccttctgttcctttatttgcccgtagtgttagtgaagattgtgaagtggcaggttacagagttctaaaaggcactgaagccgtcatcattccctatgcattgcacagagatccgagatacttccccaaccccgaggagttccagcctgagcggttcttccccgagaatgcacaagggcgccatccatatgcctacgtgcccttctctgctggccccaggaactgtataggtcaaaagtttgctgtgatggaagaaaagaccattctttcgtgcatcctgaggcacttttggatagaatccaaccagaaaagagaagagcttggtctagaaggacagttgattcttcgtccaagtaatggcatctggatcaagttgaagaggagaaatgcagatgaacgcggaagcggagctactaacttcagcctgctgaagcaggctggagacgtggaggagaaccctggacctatgggagtcaaagttctgtttgccctgatctgcatcgctgtggccgaggccgcctccctgttctctggccgcatcctgatccgcaacaatagcgaccaggacgagctggatacggaggctgaggtcagtcgcaggctggagaaccggctggtgctgctgttctttggtgctggggcttgtccacagtgccaggccttcgtgcccatcctcaaggacttcttcgtgcggctcacagatgagttctatgtactgcgggcggctcagctggccctggtgtacgtgtcccaggactccacggaggagcagcaggacctgttcctcaaggacatgccaaagaaatggcttttcctgccctttgaggatgatctgaggaggtgataaacgcgtggtttatccgatccaccggatctagataagatatccgatccaccggatctagataactgatcataatcagccataccacatttgtagaggttttacttgctttaaaaaacctcccacacctccccctgaacctgaaacataaaatgaatgcaattggcggccgcctcgagctgtgccttctagttgccagccatctgttgtttgcccctcccccgtgccttccttgaccctggaaggtgccactcccactgtcctttcctaataaaatgaggaaattgcatcgcattgtctgagtaggtgtcattctattctggggggtggggtggggcaggacagcaagggggaggattgggaagacaatagcaggcatgctggggatgcggtgggctctatgg

SEQ ID NO: 48 - protein, 126 aa, 人工序列（Artificial Sequence）
  spGL-RdCVF
MGVKVLFALICIAVAEAMASLFSGRILIRNNSDQDELDTEAEVSRRLENRLVLLFFGAGACPQCQAFVPILKDFFVRLTDEFYVLRAAQLALVYVSQDSTEEQQDLFLKDMPKKWLFLPFEDDLRR

SEQ ID NO: 49 - protein, 160 aa, 人工序列（Artificial Sequence）
  spGUCY2D-RdCVF
MTACARRAGGLPDPGLCGPAWWAPSLPRLPRALPRLPLLLLLLLLQPPALSMASLFSGRILIRNNSDQDELDTEAEVSRRLENRLVLLFFGAGACPQCQAFVPILKDFFVRLTDEFYVLRAAQLALVYVSQDSTEEQQDLFLKDMPKKWLFLPFEDDLRR

SEQ ID NO: 50 - protein, 132 aa, 人工序列（Artificial Sequence）
  spRS1-RdCVF
MSRKIEGFLLLLLFGYEATLGLSMASLFSGRILIRNNSDQDELDTEAEVSRRLENRLVLLFFGAGACPQCQAFVPILKDFFVRLTDEFYVLRAAQLALVYVSQDSTEEQQDLFLKDMPKKWLFLPFEDDLRR

SEQ ID NO: 51 - protein, 133 aa, 人工序列（Artificial Sequence）
  spNDP -RdCVF
MRKHVLAASFSMLSLLVIMGDTDSMASLFSGRILIRNNSDQDELDTEAEVSRRLENRLVLLFFGAGACPQCQAFVPILKDFFVRLTDEFYVLRAAQLALVYVSQDSTEEQQDLFLKDMPKKWLFLPFEDDLRR

SEQ ID NO: 52 - protein, 139 aa, 人工序列（Artificial Sequence）
  spGAS6-RdCVF
MAPSLSPGPAALRRAPQLLLLLLAAECALAMASLFSGRILIRNNSDQDELDTEAEVSRRLENRLVLLFFGAGACPQCQAFVPILKDFFVRLTDEFYVLRAAQLALVYVSQDSTEEQQDLFLKDMPKKWLFLPFEDDLRR

SEQ ID NO: 53 - protein, 136 aa, 人工序列（Artificial Sequence）
  spCRB1-RdCVF
MALKNINYLLIFYLSFSLLIYIKNSFCMASLFSGRILIRNNSDQDELDTEAEVSRRLENRLVLLFFGAGACPQCQAFVPILKDFFVRLTDEFYVLRAAQLALVYVSQDSTEEQQDLFLKDMPKKWLFLPFEDDLRR

SEQ ID NO: 54 - protein, 137 aa, 人工序列（Artificial Sequence）
  spCRB2-RdCVF
MALARPGTPDPQALASVLLLLLWAPALSMASLFSGRILIRNNSDQDELDTEAEVSRRLENRLVLLFFGAGACPQCQAFVPILKDFFVRLTDEFYVLRAAQLALVYVSQDSTEEQQDLFLKDMPKKWLFLPFEDDLRR

SEQ ID NO: 55 - protein, 651 aa, 人工序列（Artificial Sequence）
  CYP4V2-spGL-RdCVF
MAGLWLGLVWQKLLLWGAASALSLAGASLVLSLLQRVASYARKWQQMRPIPTVARAYPLVGHALLMKPDGREFFQQIIEYTEEYRHMPLLKLWVGPVPMVALYNAENVEVILTSSKQIDKSSMYKFLEPWLGLGLLTSTGNKWRSRRKMLTPTFHFTILEDFLDIMNEQANILVKKLEKHINQEAFNCFFYITLCALDIICETAMGKNIGAQSNDDSEYVRAVYRMSEMIFRRIKMPWLWLDLWYLMFKEGWEHKKSLQILHTFTNSVIAERANEMNANEDCRGDGRGSAPSKNKRRAFLDLLLSVTDDEGNRLSHEDIREEVDTFMFEGHDTTAAAINWSLYLLGSNPEVQKKVDHELDDVFGKSDRPATVEDLKKLRYLECVIKETLRLFPSVPLFARSVSEDCEVAGYRVLKGTEAVIIPYALHRDPRYFPNPEEFQPERFFPENAQGRHPYAYVPFSAGPRNCIGQKFAVMEEKTILSCILRHFWIESNQKREELGLEGQLILRPSNGIWIKLKRRNADERMGVKVLFALICIAVAEAMASLFSGRILIRNNSDQDELDTEAEVSRRLENRLVLLFFGAGACPQCQAFVPILKDFFVRLTDEFYVLRAAQLALVYVSQDSTEEQQDLFLKDMPKKWLFLPFEDDLRR